European Patent Specification EP 3 510 049 B1, published November 8, 2023. Title: ACID-ALPHA GLUCOSIDASE VARIANTS AND USES THEREOF. Applicant: GENETHON et al. The sequence listing filed with the application follows.

SEQUENCE LISTING (54 sequences)

SEQ ID NO: 1 - DNA, 2859 bp, homo sapiens
atgggagtgaggcacccgccctgctcccaccggctcctggccgtctgcgccctcgtgtccttggcaaccgcagcgctcctggggcacatcctactccatgatttcctgctggttccccgagagctgagtggctcctccccagtcctggaggagactcacccagctcaccagcagggagccagcagaccagggccccgggatgcccaggcacaccccgggcggccgcgagcagtgcccacacagtgcgacgtcccccccaacagccgcttcgattgcgcccctgacaaggccatcacccaggaacagtgcgaggcccgcggctgttgctacatccctgcaaagcaggggctgcagggagcccagatggggcagccctggtgcttcttcccacccagctaccccagctacaagctggagaacctgagctcctctgaaatgggctacacggccaccctgacccgtaccacccccaccttcttccccaaggacatcctgaccctgcggctggacgtgatgatggagactgagaaccgcctccacttcacgatcaaagatccagctaacaggcgctacgaggtgcccttggagaccccgcatgtccacagccgggcaccgtccccactctacagcgtggagttctccgaggagcccttcggggtgatcgtgcgccggcagctggacggccgcgtgctgctgaacacgacggtggcgcccctgttctttgcggaccagttccttcagctgtccacctcgctgccctcgcagtatatcacaggcctcgccgagcacctcagtcccctgatgctcagcaccagctggaccaggatcaccctgtggaaccgggaccttgcgcccacgcccggtgcgaacctctacgggtctcaccctttctacctggcgctggaggacggcgggtcggcacacggggtgttcctgctaaacagcaatgccatggatgtggtcctgcagccgagccctgcccttagctggaggtcgacaggtgggatcctggatgtctacatcttcctgggcccagagcccaagagcgtggtgcagcagtacctggacgttgtgggatacccgttcatgccgccatactggggcctgggcttccacctgtgccgctggggctactcctccaccgctatcacccgccaggtggtggagaacatgaccagggcccacttccccctggacgtccagtggaacgacctggactacatggactcccggagggacttcacgttcaacaaggatggcttccgggacttcccggccatggtgcaggagctgcaccagggcggccggcgctacatgatgatcgtggatcctgccatcagcagctcgggccctgccgggagctacaggccctacgacgagggtctgcggaggggggttttcatcaccaacgagaccggccagccgctgattgggaaggtatggcccgggtccactgccttccccgacttcaccaaccccacagccctggcctggtgggaggacatggtggctgagttccatgaccaggtgcccttcgacggcatgtggattgacatgaacgagccttccaacttcatcaggggctctgaggacggctgccccaacaatgagctggagaacccaccctacgtgcctggggtggttggggggaccctccaggcggccaccatctgtgcctccagccaccagtttctctccacacactacaacctgcacaacctctacggcctgaccgaagccatcgcctcccacagggcgctggtgaaggctcgggggacacgcccatttgtgatctcccgctcgacctttgctggccacggccgatacgccggccactggacgggggacgtgtggagctcctgggagcagctcgcctcctccgtgccagaaatcctgcagtttaacctgctgggggtgcctctggtcggggccgacgtctgcggcttcctgggcaacacctcagaggagctgtgtgtgcgctggacccagctgggggccttctaccccttcatgcggaaccacaacagcctgctcagtctgccccaggagccgtacagcttcagcgagccggcccagcaggccatgaggaaggccctcaccctgcgctacgcactcctcccccacctctacacactgttccaccaggcccacgtcgcgggggagaccgtggcccggcccctcttcctggagttccccaaggactctagcacctggactgtggaccaccagctcctgtggggggaggccctgctcatcaccccagtgctccaggccgggaaggccgaagtgactggctacttccccttgggcacatggtacgacctgcagacggtgccagtagaggcccttggcagcctcccacccccacctgcagctccccgtgagccagccatccacagcgaggggcagtgggtgacgctgccggcccccctggacaccatcaacgtccacctccgggctgggtacatcatccccctgcagggccctggcctcacaaccacagagtcccgccagcagcccatggccctggctgtggccctgaccaagggtggggaggcccgaggggagctgttctgggacgatggagagagcctggaagtgctggagcgaggggcctacacacaggtcatcttcctggccaggaataacacgatcgtgaatgagctggtacgtgtgaccagtgagggagctggcctgcagctgcagaaggtgactgtcctgggcgtggccacggcgccccagcaggtcctctccaacggtgtccctgtctccaacttcacctacagccccgacaccaaggtcctggacatctgtgtctcgctgttgatgggagagcagtttctcgtcagctggtgttag

SEQ ID NO: 2 - protein, 18 aa, artificial
  sp7
MAFLWLLSCWALLGTTFG

SEQ ID NO: 3 - protein, 25 aa, artificial
  sp6
MPPPRTGRGLLWLGLVLSSVCVALG

SEQ ID NO: 4 - protein, 22 aa, artificial
  sp8
MASRLTLLTLLLLLLAGDRASS

SEQ ID NO: 5 - protein, 925 aa, artificial
  hGAAwt w/o sp
GHILLHDFLLVPRELSGSSPVLEETHPAHQQGASRPGPRDAQAHPGRPRAVPTQCDVPPNSRFDCAPDKAITQEQCEARGCCYIPAKQGLQGAQMGQPWCFFPPSYPSYKLENLSSSEMGYTATLTRTTPTFFPKDILTLRLDVMMETENRLHFTIKDPANRRYEVPLETPHVHSRAPSPLYSVEFSEEPFGVIVRRQLDGRVLLNTTVAPLFFADQFLQLSTSLPSQYITGLAEHLSPLMLSTSWTRITLWNRDLAPTPGANLYGSHPFYLALEDGGSAHGVFLLNSNAMDVVLQPSPALSWRSTGGILDVYIFLGPEPKSVVQQYLDVVGYPFMPPYWGLGFHLCRWGYSSTAITRQVVENMTRAHFPLDVQWNDLDYMDSRRDFTFNKDGFRDFPAMVQELHQGGRRYMMIVDPAISSSGPAGSYRPYDEGLRRGVFITNETGQPLIGKVWPGSTAFPDFTNPTALAWWEDMVAEFHDQVPFDGMWIDMNEPSNFIRGSEDGCPNNELENPPYVPGVVGGTLQAATICASSHQFLSTHYNLHNLYGLTEAIASHRALVKARGTRPFVISRSTFAGHGRYAGHWTGDVWSSWEQLASSVPEILQFNLLGVPLVGADVCGFLGNTSEELCVRWTQLGAFYPFMRNHNSLLSLPQEPYSFSEPAQQAMRKALTLRYALLPHLYTLFHQAHVAGETVARPLFLEFPKDSSTWTVDHQLLWGEALLITPVLQAGKAEVTGYFPLGTWYDLQTVPVEALGSLPPPPAAPREPAIHSEGQWVTLPAPLDTINVHLRAGYIIPLQGPGLTTTESRQQPMALAVALTKGGEARGELFWDDGESLEVLERGAYTQVIFLARNNTIVNELVRVTSEGAGLQLQKVTVLGVATAPQQVLSNGVPVSNFTYSPDTKVLDICVSLLMGEQFLVSWC

SEQ ID NO: 6 - DNA, 441 bp, artificial
  HBB2 intron
gtacacatattgaccaaatcagggtaattttgcatttgtaattttaaaaaatgctttcttcttttaatatacttttttgtttatcttatttctaatactttccctaatctctttctttcagggcaataatgatacaatgtatcatgcctctttgcaccattctaaagaataacagtgataatttctgggttaaggcaatagcaatatttctgcatataaatatttctgcatataaattgtaactgatgtaagaggtttcatattgctaatagcagctacaatccagctaccattctgcttttattttatggttgggataaggctggattattctgagtccaagctaggcccttttgctaatcatgttcatacctcttatcttcctcccacagctcctgggcaacgtgctggtctgtgtgctggcccatcactttggcaaag

SEQ ID NO: 7 - DNA, 441 bp, modified HBB2 intron
gtacacatattgaccaaatcagggtaattttgcatttgtaattttaaaaaatgctttcttcttttaatatacttttttgtttatcttatttctaatactttccctaatctctttctttcagggcaataatgatacaatgtatcatgcctctttgcaccattctaaagaataacagtgataatttctgggttaaggcaatagcaatatttctgcatataaatatttctgcatataaattgtaactgatgtaagaggtttcatattgctaatagcagctacaatccagctaccattctgcttttattttctggttgggataaggctggattattctgagtccaagctaggcccttttgctaatcttgttcatacctcttatcttcctcccacagctcctgggcaacctgctggtctctctgctggcccatcactttggcaaag

SEQ ID NO: 8 - DNA, 1438 bp, artificial
  FIX intron
ggtttgtttccttttttaaaatacattgagtatgcttgccttttagatatagaaatatctgatgctgtcttcttcactaaattttgattacatgatttgacagcaatattgaagagtctaacagccagcacgcaggttggtaagtactggttctttgttagctaggttttcttcttcttcatttttaaaactaaatagatcgacaatgcttatgatgcatttatgtttaataaacactgttcagttcatgatttggtcatgtaattcctgttagaaaacattcatctccttggtttaaaaaaattaaaagtgggaaaacaaagaaatagcagaatatagtgaaaaaaaataaccacattatttttgtttggacttaccactttgaaatcaaaatgggaaacaaaagcacaaacaatggccttatttacacaaaaagtctgattttaagatatatgacatttcaaggtttcagaagtatgtaatgaggtgtgtctctaattttttaaattatatatcttcaatttaaagttttagttaaaacataaagattaacctttcattagcaagctgttagttatcaccaacgcttttcatggattaggaaaaaatcattttgtctctatgtcaaacatcttggagttgatatttggggaaacacaatactcagttgagttccctaggggagaaaagcacgcttaagaattgacataaagagtaggaagttagctaatgcaacatatatcactttgttttttcacaactacagtgactttatgtatttcccagaggaaggcatacagggaagaaattatcccatttggacaaacagcatgttctcacaggaagcatttatcacacttacttgtcaactttctagaatcaaatctagtagctgacagtaccaggatcaggggtgccaaccctaagcacccccagaaagctgactggccctgtggttcccactccagacatgatgtcagctgtgaaatcgacgtcgctggaccataattaggcttctgttcttcaggagacatttgttcaaagtcatttgggcaaccatattctgaaaacagcccagccagggtgatggatcactttgcaaagatcctcaatgagctattttcaagtgatgacaaagtgtgaagttaaccgctcatttgagaactttctttttcatccaaagtaaattcaaatatgattagaaatctgaccttttattactggaattctcttgactaaaagtaaaattgaattttaattcctaaatctccatgtgtatacagtactgtgggaacatcacagattttggctccatgccctaaagagaaattggctttcagattatttggattaaaaacaaagactttcttaagagatgtaaaattttcatgatgttttcttttttgctaaaactaaagaattattcttttacatttca

SEQ ID NO: 9 - DNA, 1438 bp, artificial
  modified FIX intron
ggtttgtttccttttttaaaatacattgagtatgcttgccttttagatatagaaatatctgatgctgtcttcttcactaaattttgattacatgatttgacagcaatattgaagagtctaacagccagcacgcaggttggtaagtactggttctttgttagctaggttttcttcttcttcatttttaaaactaaatagatcgacattgcttttgttgcatttatgtttaataaacactgttcagttcatgatttggtcatgtaattcctgttagaaaacattcatctccttggtttaaaaaaattaaaagtgggaaaacaaagaaatagcagaatatagtgaaaaaaaataaccacattatttttgtttggacttaccactttgaaatcaaattgggaaacaaaagcacaaacaatggccttatttacacaaaaagtctgattttaagatatatgacatttcaaggtttcagaagtatgtaatgaggtgtgtctctaattttttaaattatatatcttcaatttaaagttttagttaaaacataaagattaacctttcattagcaagctgttagttatcaccaacgcttttcatggattaggaaaaaatcattttgtctctttgtcaaacatcttggagttgatatttggggaaacacaatactcagttgagttccctaggggagaaaagcacgcttaagaattgacataaagagtaggaagttagctattgcaacatatatcactttgttttttcacaactacagtgactttttgtatttcccagaggaaggcatacagggaagaaattatcccatttggacaaacagcttgttctcacaggaagcatttatcacacttacttgtcaactttctagaatcaaatctagtagctgacagtaccaggatcaggggtgccaaccctaagcacccccagaaagctgactggccctgtggttcccactccagacatgatgtcagctgtgaaatcgacgtcgctggaccataattaggcttctgttcttcaggagacatttgttcaaagtcatttgggcaaccatattctgaaaacagcccagccagggtgttggatcactttgcaaagatcctcattgagctattttcaagtgttgacaaagtgtgaagttaaccgctcatttgagaactttctttttcatccaaagtaaattcaaatatgattagaaatctgaccttttattactggaattctcttgactaaaagtaaaattgaattttaattcctaaatctccatgtgtatacagtactgtgggaacatcacagattttggctccatgccctaaagagaaattggctttcagattatttggattaaaaacaaagactttcttaagagatgtaaaattttcttgttgttttcttttttgctaaaactaaagaattattcttttacatttca

SEQ ID NO: 10 - DNA, 881 bp, artificial
  chicken beta-globin intron
gcgggagtcgctgcgttgccttcgccccgtgccccgctccgccgccgcctcgcgccgcccgccccggctctgactgaccgcgttactcccacaggtgagcgggcgggacggcccttctcctccgggctgtaattagcgcttggtttaatgacggcttgtttcttttctgtggctgcgtgaaagccttgaggggctccgggagggccctttgtgcggggggagcggctcggggggtgcgtgcgtgtgtgtgtgcgtggggagcgccgcgtgcggctccgcgctgcccggcggctgtgagcgctgcgggcgcggcgcggggctttgtgcgctccgcagtgtgcgcgaggggagcgcggccgggggcggtgccccgcggtgcggggggggctgcgaggggaacaaaggctgcgtgcggggtgtgtgcgtgggggggtgagcagggggtgtgggcgcgtcggtcgggctgcaaccccccctgcacccccctccccgagttgctgagcacggcccggcttcgggtgcggggctccgtacggggcgtggcgcggggctcgccgtgccgggcggggggtggcggcaggtgggggtgccgggcggggcggggccgcctcgggccggggagggctcgggggaggggcgcggcggcccccggagcgccggcggctgtcgaggcgcggcgagccgcagccattgccttttatggtaatcgtgcgagagggcgcagggacttcctttgtcccaaatctgtgcggagccgaaatctgggaggcgccgccgcaccccctctagcgggcgcggggcgaagcggtgcggcgccggcaggaaggaaatgggcggggagggccttcgtgcgtcgccgcgccgccgtccccttctccctc

SEQ ID NO: 11 - DNA, 881 bp, artificial
  modified chicken beta-globin intron
gcgggagtcgctgcgttgccttcgccccgtgccccgctccgccgccgcctcgcgccgcccgccccggctctgactgaccgcgttactcccacaggtgagcgggcgggacggcccttctcctccgggctgtaattagcgcttggtttaatgacggcttgtttcttttctgtggctgcgtgaaagccttgaggggctccgggagggccctttgtgcggggggagcggctcggggggtgcgtgcgtgtgtgtgtgcgtggggagcgccgcgtgcggctccgcgctgcccggcggctgtgagcgctgcgggcgcggcgcggggctttgtgcgctccgcagtgtgcgcgaggggagcgcggccgggggcggtgccccgcggtgcggggggggctgcgaggggaacaaaggctgcgtgcggggtgtgtgcgtgggggggtgagcagggggtgtgggcgcgtcggtcgggctgcaaccccccctgcacccccctccccgagttgctgagcacggcccggcttcgggtgcggggctccgtacggggcgtggcgcggggctcgccgtgccgggcggggggtggcggcaggtgggggtgccgggcggggcggggccgcctcgggccggggagggctcgggggaggggcgcggcggcccccggagcgccggcggctgtcgaggcgcggcgagccgcagccattgccttttttggtaatcgtgcgagagggcgcagggacttcctttgtcccaaatctgtgcggagccgaaatctgggaggcgccgccgcaccccctctagcgggcgcggggcgaagcggtgcggcgccggcaggaaggaattgggcggggagggccttcgtgcgtcgccgcgccgccgtccccttctccctc

SEQ ID NO: 12 - protein, 952 aa, homo sapiens
MGVRHPPCSHRLLAVCALVSLATAALLGHILLHDFLLVPRELSGSSPVLEETHPAHQQGASRPGPRDAQAHPGRPRAVPTQCDVPPNSRFDCAPDKAITQEQCEARGCCYIPAKQGLQGAQMGQPWCFFPPSYPSYKLENLSSSEMGYTATLTRTTPTFFPKDILTLRLDVMMETENRLHFTIKDPANRRYEVPLETPHVHSRAPSPLYSVEFSEEPFGVIVRRQLDGRVLLNTTVAPLFFADQFLQLSTSLPSQYITGLAEHLSPLMLSTSWTRITLWNRDLAPTPGANLYGSHPFYLALEDGGSAHGVFLLNSNAMDVVLQPSPALSWRSTGGILDVYIFLGPEPKSVVQQYLDVVGYPFMPPYWGLGFHLCRWGYSSTAITRQVVENMTRAHFPLDVQWNDLDYMDSRRDFTFNKDGFRDFPAMVQELHQGGRRYMMIVDPAISSSGPAGSYRPYDEGLRRGVFITNETGQPLIGKVWPGSTAFPDFTNPTALAWWEDMVAEFHDQVPFDGMWIDMNEPSNFIRGSEDGCPNNELENPPYVPGVVGGTLQAATICASSHQFLSTHYNLHNLYGLTEAIASHRALVKARGTRPFVISRSTFAGHGRYAGHWTGDVWSSWEQLASSVPEILQFNLLGVPLVGADVCGFLGNTSEELCVRWTQLGAFYPFMRNHNSLLSLPQEPYSFSEPAQQAMRKALTLRYALLPHLYTLFHQAHVAGETVARPLFLEFPKDSSTWTVDHQLLWGEALLITPVLQAGKAEVTGYFPLGTWYDLQTVPVEALGSLPPPPAAPREPAIHSEGQWVTLPAPLDTINVHLRAGYIIPLQGPGLTTTESRQQPMALAVALTKGGEARGELFWDDGESLEVLERGAYTQVIFLARNNTIVNELVRVTSEGAGLQLQKVTVLGVATAPQQVLSNGVPVSNFTYSPDTKVLDICVSLLMGEQFLVSWC

SEQ ID NO: 13 - DNA, 2778 bp, artificial
  hGAAco1 w/o sp
ggccatatcctgctgcacgactttctactagtgcccagagagctgagcggcagctctcccgtgctggaagaaacacaccctgcccatcagcagggcgcctctagacctggacctagagatgcccaggcccaccccggcagacctagagctgtgcctacccagtgtgacgtgccccccaacagcagattcgactgcgcccctgacaaggccatcacccaggaacagtgcgaggccagaggctgctgctacatccctgccaagcagggactgcagggcgctcagatgggacagccctggtgcttcttcccaccctcctaccccagctacaagctggaaaacctgagcagcagcgagatgggctacaccgccaccctgaccagaaccacccccacattcttcccaaaggacatcctgaccctgcggctggacgtgatgatggaaaccgagaaccggctgcacttcaccatcaaggaccccgccaatcggagatacgaggtgcccctggaaaccccccacgtgcactctagagcccccagccctctgtacagcgtggaattcagcgaggaacccttcggcgtgatcgtgcggagacagctggatggcagagtgctgctgaacaccaccgtggcccctctgttcttcgccgaccagttcctgcagctgagcaccagcctgcccagccagtacatcacaggactggccgagcacctgagccccctgatgctgagcacatcctggacccggatcaccctgtggaacagggatctggcccctacccctggcgccaatctgtacggcagccaccctttctacctggccctggaagatggcggatctgcccacggagtgtttctgctgaactccaacgccatggacgtggtgctgcagcctagccctgccctgtcttggagaagcacaggcggcatcctggatgtgtacatctttctgggccccgagcccaagagcgtggtgcagcagtatctggatgtcgtgggctaccccttcatgcccccttactggggcctgggattccacctgtgcagatggggctactccagcaccgccatcaccagacaggtggtggaaaacatgaccagagcccacttcccactggatgtgcagtggaacgacctggactacatggacagcagacgggacttcaccttcaacaaggacggcttccgggacttccccgccatggtgcaggaactgcatcagggcggcagacggtacatgatgatcgtggatcccgccatcagctcctctggccctgccggctcttacagaccctacgacgagggcctgcggagaggcgtgttcatcaccaacgagacaggccagcccctgatcggcaaagtgtggcctggcagcacagccttccccgacttcaccaatcctaccgccctggcttggtgggaggacatggtggccgagttccacgaccaggtgcccttcgacggcatgtggatcgacatgaacgagcccagcaacttcatccggggcagcgaggatggctgccccaacaacgaactggaaaatcccccttacgtgcccggcgtcgtgggcggaacactgcaggccgctacaatctgtgccagcagccaccagtttctgagcacccactacaacctgcacaacctgtacggcctgaccgaggccattgccagccaccgcgctctcgtgaaagccagaggcacacggcccttcgtgatcagcagaagcacctttgccggccacggcagatacgccggacattggactggcgacgtgtggtcctcttgggagcagctggcctctagcgtgcccgagatcctgcagttcaatctgctgggcgtgccactcgtgggcgccgatgtgtgtggcttcctgggcaacacctccgaggaactgtgtgtgcggtggacacagctgggcgccttctaccctttcatgagaaaccacaacagcctgctgagcctgccccaggaaccctacagctttagcgagcctgcacagcaggccatgcggaaggccctgacactgagatacgctctgctgccccacctgtacaccctgtttcaccaggcccatgtggccggcgagacagtggccagacctctgtttctggaattccccaaggacagcagcacctggaccgtggaccatcagctgctgtggggagaggctctgctgattaccccagtgctgcaggcaggcaaggccgaagtgaccggctactttcccctgggcacttggtacgacctgcagaccgtgcctgtggaagccctgggatctctgcctccacctcctgccgctcctagagagcctgccattcactctgagggccagtgggtcacactgcctgcccccctggataccatcaacgtgcacctgagggccggctacatcataccactgcagggacctggcctgaccaccaccgagtctagacagcagccaatggccctggccgtggccctgaccaaaggcggagaagctaggggcgagctgttctgggacgatggcgagagcctggaagtgctggaaagaggcgcctatacccaagtgatcttcctggcccggaacaacaccatcgtgaacgagctggtgcgcgtgacctctgaaggcgctggactgcagctgcagaaagtgaccgtgctgggagtggccacagcccctcagcaggtgctgtctaatggcgtgcccgtgtccaacttcacctacagccccgacaccaaggtgctggacatctgcgtgtcactgctgatgggagagcagtttctggtgtcctggtgctga

SEQ ID NO: 14 - DNA, 2778 bp, artificial
  hGAAco2 w/o sp
ggacacatcctgctgcacgacttcctgttggtgcctagagagctgagcggatcatccccagtgctggaggagactcatcctgctcaccaacagggagcttccagaccaggaccgagagacgcccaagcccatcctggtagaccaagagctgtgcctacccaatgcgacgtgccacccaactcccgattcgactgcgcgccagataaggctattacccaagagcagtgtgaagccagaggttgctgctacatcccagcgaagcaaggattgcaaggcgcccaaatgggacaaccttggtgtttcttccccccttcgtacccatcatataaactcgaaaacctgtcctcttcggaaatgggttatactgccaccctcaccagaactactcctactttcttcccgaaagacatcttgaccttgaggctggacgtgatgatggagactgaaaaccggctgcatttcactatcaaagatcctgccaatcggcgatacgaggtccctctggaaacccctcacgtgcactcacgggctccttctccgctttactccgtcgaattctctgaggaacccttcggagtgatcgttagacgccagctggatggtagagtgctgttgaacactactgtggccccacttttcttcgctgaccagtttctgcaactgtccacttccctgccatcccagtacattactggactcgccgaacacctgtcgccactgatgctctcgacctcttggactagaatcactttgtggaacagagacttggcccctactccgggagcaaatctgtacggaagccaccctttttacctggcgctcgaagatggcggatccgctcacggagtgttcctgctgaatagcaacgcaatggacgtggtgctgcaaccttcccctgcactcagttggagaagtaccgggggtattctggacgtgtacatcttcctcggaccagaacccaagagcgtggtgcagcaatatctggacgtggtcggatacccttttatgcctccttactggggactgggattccacctttgccgttggggctactcatccaccgccattaccagacaggtggtggagaatatgaccagagcccacttccctctcgacgtgcagtggaacgatctggactatatggactcccggagagatttcaccttcaacaaggacgggttccgcgattttcccgcgatggttcaagagctccaccagggtggtcgaagatatatgatgatcgtcgacccagccatttcgagcagcggacccgctggatcttatagaccttacgacgaaggccttaggagaggagtgttcatcacaaacgagactggacagcctttgatcggtaaagtgtggcctggatcaaccgcctttcctgactttaccaatcccactgccttggcttggtgggaggacatggtggccgaattccacgaccaagtcccctttgatggaatgtggatcgatatgaacgaaccaagcaattttatcagaggttccgaagacggttgccccaacaacgaactggaaaaccctccttatgtgcccggagtcgtgggcggaacattacaggccgcgactatttgcgccagcagccaccaattcctgtccactcactacaacctccacaacctttatggattaaccgaagctattgcaagtcacagggctctggtgaaggctagagggactaggccctttgtgatctcccgatccacctttgccggacacgggagatacgccggtcactggactggtgacgtgtggagctcatgggaacaactggcctcctccgtgccggaaatcttacagttcaaccttctgggtgtccctcttgtcggagcagacgtgtgtgggtttcttggtaacacctccgaggaactgtgtgtgcgctggactcaactgggtgcattctacccattcatgagaaaccacaactccttgctgtccctgccacaagagccctactcgttcagcgagcctgcacaacaggctatgcggaaggcactgaccctgagatacgccctgcttccacacttatacactctcttccatcaagcgcatgtggcaggagaaaccgttgcaaggcctcttttccttgaattccccaaggattcctcgacttggacggtggatcatcagctgctgtggggagaagctctgctgattactccagtgttgcaagccggaaaagctgaggtgaccggatactttccgctgggaacctggtacgacctccagactgtccctgttgaagcccttggatcactgcctccgcctccggcagctccacgcgaaccagctatacattccgagggacagtgggttacattaccagctcctctggacacaatcaacgtccacttaagagctggctacattatccctctgcaaggaccaggactgactacgaccgagagcagacagcagccaatggcactggctgtggctctgaccaagggaggggaagctagaggagaactcttctgggatgatggggagtcccttgaagtgctggaaagaggcgcttacactcaagtcattttccttgcacggaacaacaccattgtgaacgaattggtgcgagtgaccagcgaaggagctggacttcaactgcagaaggtcactgtgctcggagtggctaccgctcctcagcaagtgctgtcgaatggagtccccgtgtcaaactttacctactcccctgacactaaggtgctcgacatttgcgtgtccctcctgatgggagagcagttccttgtgtcctggtgttga

SEQ ID NO: 15 - DNA, 397 bp, artificial
  hAAT promoter
gatcttgctaccagtggaacagccactaaggattctgcagtgagagcagagggccagctaagtggtactctcccagagactgtctgactcacgccaccccctccaccttggacacaggacgctgtggtttctgagccaggtacaatgactcctttcggtaagtgcagtggaagctgtacactgcccaggcaaagcgtccgggcagcgtaggcgggcgactcagatcccagccagtggacttagcccctgtttgctcctccgataactggggtgaccttggttaatattcaccagcagcctcccccgttgcccctctggatccactgcttaaatacggacgaggacagggccctgtctcctcagcttcaggcaccaccactgacctgggacagtgaat

SEQ ID NO: 16 - DNA, 321 bp, artificial
  ApoE control region
aggctcagaggcacacaggagtttctgggctcaccctgcccccttccaacccctcagttcccatcctccagcagctgtttgtgtgctgcctctgaagtccacactgaacaaacttcagcctactcatgtccctaaaatgggcaaacattgcaagcagcaaacagcaaacacacagccctccctgcctgctgaccttggagctggggcagaggtcagagacctctctgggcccatgccacctccaacatccactcgaccccttggaatttcggtggagaggagcagaggttgtcctggcgtggtttaggtagtgtgagaggg

SEQ ID NO: 17 - DNA, 2808 bp, artificial
  sp7+hGAAco1-delta-8
atggcctttctgtggctgctgagctgttgggccctgctgggcaccaccttcggcctactagtgcccagagagctgagcggcagctctcccgtgctggaagaaacacaccctgcccatcagcagggcgcctctagacctggacctagagatgcccaggcccaccccggcagacctagagctgtgcctacccagtgtgacgtgccccccaacagcagattcgactgcgcccctgacaaggccatcacccaggaacagtgcgaggccagaggctgctgctacatccctgccaagcagggactgcagggcgctcagatgggacagccctggtgcttcttcccaccctcctaccccagctacaagctggaaaacctgagcagcagcgagatgggctacaccgccaccctgaccagaaccacccccacattcttcccaaaggacatcctgaccctgcggctggacgtgatgatggaaaccgagaaccggctgcacttcaccatcaaggaccccgccaatcggagatacgaggtgcccctggaaaccccccacgtgcactctagagcccccagccctctgtacagcgtggaattcagcgaggaacccttcggcgtgatcgtgcggagacagctggatggcagagtgctgctgaacaccaccgtggcccctctgttcttcgccgaccagttcctgcagctgagcaccagcctgcccagccagtacatcacaggactggccgagcacctgagccccctgatgctgagcacatcctggacccggatcaccctgtggaacagggatctggcccctacccctggcgccaatctgtacggcagccaccctttctacctggccctggaagatggcggatctgcccacggagtgtttctgctgaactccaacgccatggacgtggtgctgcagcctagccctgccctgtcttggagaagcacaggcggcatcctggatgtgtacatctttctgggccccgagcccaagagcgtggtgcagcagtatctggatgtcgtgggctaccccttcatgcccccttactggggcctgggattccacctgtgcagatggggctactccagcaccgccatcaccagacaggtggtggaaaacatgaccagagcccacttcccactggatgtgcagtggaacgacctggactacatggacagcagacgggacttcaccttcaacaaggacggcttccgggacttccccgccatggtgcaggaactgcatcagggcggcagacggtacatgatgatcgtggatcccgccatcagctcctctggccctgccggctcttacagaccctacgacgagggcctgcggagaggcgtgttcatcaccaacgagacaggccagcccctgatcggcaaagtgtggcctggcagcacagccttccccgacttcaccaatcctaccgccctggcttggtgggaggacatggtggccgagttccacgaccaggtgcccttcgacggcatgtggatcgacatgaacgagcccagcaacttcatccggggcagcgaggatggctgccccaacaacgaactggaaaatcccccttacgtgcccggcgtcgtgggcggaacactgcaggccgctacaatctgtgccagcagccaccagtttctgagcacccactacaacctgcacaacctgtacggcctgaccgaggccattgccagccaccgcgctctcgtgaaagccagaggcacacggcccttcgtgatcagcagaagcacctttgccggccacggcagatacgccggacattggactggcgacgtgtggtcctcttgggagcagctggcctctagcgtgcccgagatcctgcagttcaatctgctgggcgtgccactcgtgggcgccgatgtgtgtggcttcctgggcaacacctccgaggaactgtgtgtgcggtggacacagctgggcgccttctaccctttcatgagaaaccacaacagcctgctgagcctgccccaggaaccctacagctttagcgagcctgcacagcaggccatgcggaaggccctgacactgagatacgctctgctgccccacctgtacaccctgtttcaccaggcccatgtggccggcgagacagtggccagacctctgtttctggaattccccaaggacagcagcacctggaccgtggaccatcagctgctgtggggagaggctctgctgattaccccagtgctgcaggcaggcaaggccgaagtgaccggctactttcccctgggcacttggtacgacctgcagaccgtgcctgtggaagccctgggatctctgcctccacctcctgccgctcctagagagcctgccattcactctgagggccagtgggtcacactgcctgcccccctggataccatcaacgtgcacctgagggccggctacatcataccactgcagggacctggcctgaccaccaccgagtctagacagcagccaatggccctggccgtggccctgaccaaaggcggagaagctaggggcgagctgttctgggacgatggcgagagcctggaagtgctggaaagaggcgcctatacccaagtgatcttcctggcccggaacaacaccatcgtgaacgagctggtgcgcgtgacctctgaaggcgctggactgcagctgcagaaagtgaccgtgctgggagtggccacagcccctcagcaggtgctgtctaatggcgtgcccgtgtccaacttcacctacagccccgacaccaaggtgctggacatctgcgtgtcactgctgatgggagagcagtttctggtgtcctggtgctga

SEQ ID NO: 18 - DNA, 2829 bp, artificial
  sp6+hGAAco1-delta-8
atgcctccacctagaacaggcagaggcctgctgtggctgggcctggtgctgtctagtgtgtgtgtggccctgggcctactagtgcccagagagctgagcggcagctctcccgtgctggaagaaacacaccctgcccatcagcagggcgcctctagacctggacctagagatgcccaggcccaccccggcagacctagagctgtgcctacccagtgtgacgtgccccccaacagcagattcgactgcgcccctgacaaggccatcacccaggaacagtgcgaggccagaggctgctgctacatccctgccaagcagggactgcagggcgctcagatgggacagccctggtgcttcttcccaccctcctaccccagctacaagctggaaaacctgagcagcagcgagatgggctacaccgccaccctgaccagaaccacccccacattcttcccaaaggacatcctgaccctgcggctggacgtgatgatggaaaccgagaaccggctgcacttcaccatcaaggaccccgccaatcggagatacgaggtgcccctggaaaccccccacgtgcactctagagcccccagccctctgtacagcgtggaattcagcgaggaacccttcggcgtgatcgtgcggagacagctggatggcagagtgctgctgaacaccaccgtggcccctctgttcttcgccgaccagttcctgcagctgagcaccagcctgcccagccagtacatcacaggactggccgagcacctgagccccctgatgctgagcacatcctggacccggatcaccctgtggaacagggatctggcccctacccctggcgccaatctgtacggcagccaccctttctacctggccctggaagatggcggatctgcccacggagtgtttctgctgaactccaacgccatggacgtggtgctgcagcctagccctgccctgtcttggagaagcacaggcggcatcctggatgtgtacatctttctgggccccgagcccaagagcgtggtgcagcagtatctggatgtcgtgggctaccccttcatgcccccttactggggcctgggattccacctgtgcagatggggctactccagcaccgccatcaccagacaggtggtggaaaacatgaccagagcccacttcccactggatgtgcagtggaacgacctggactacatggacagcagacgggacttcaccttcaacaaggacggcttccgggacttccccgccatggtgcaggaactgcatcagggcggcagacggtacatgatgatcgtggatcccgccatcagctcctctggccctgccggctcttacagaccctacgacgagggcctgcggagaggcgtgttcatcaccaacgagacaggccagcccctgatcggcaaagtgtggcctggcagcacagccttccccgacttcaccaatcctaccgccctggcttggtgggaggacatggtggccgagttccacgaccaggtgcccttcgacggcatgtggatcgacatgaacgagcccagcaacttcatccggggcagcgaggatggctgccccaacaacgaactggaaaatcccccttacgtgcccggcgtcgtgggcggaacactgcaggccgctacaatctgtgccagcagccaccagtttctgagcacccactacaacctgcacaacctgtacggcctgaccgaggccattgccagccaccgcgctctcgtgaaagccagaggcacacggcccttcgtgatcagcagaagcacctttgccggccacggcagatacgccggacattggactggcgacgtgtggtcctcttgggagcagctggcctctagcgtgcccgagatcctgcagttcaatctgctgggcgtgccactcgtgggcgccgatgtgtgtggcttcctgggcaacacctccgaggaactgtgtgtgcggtggacacagctgggcgccttctaccctttcatgagaaaccacaacagcctgctgagcctgccccaggaaccctacagctttagcgagcctgcacagcaggccatgcggaaggccctgacactgagatacgctctgctgccccacctgtacaccctgtttcaccaggcccatgtggccggcgagacagtggccagacctctgtttctggaattccccaaggacagcagcacctggaccgtggaccatcagctgctgtggggagaggctctgctgattaccccagtgctgcaggcaggcaaggccgaagtgaccggctactttcccctgggcacttggtacgacctgcagaccgtgcctgtggaagccctgggatctctgcctccacctcctgccgctcctagagagcctgccattcactctgagggccagtgggtcacactgcctgcccccctggataccatcaacgtgcacctgagggccggctacatcataccactgcagggacctggcctgaccaccaccgagtctagacagcagccaatggccctggccgtggccctgaccaaaggcggagaagctaggggcgagctgttctgggacgatggcgagagcctggaagtgctggaaagaggcgcctatacccaagtgatcttcctggcccggaacaacaccatcgtgaacgagctggtgcgcgtgacctctgaaggcgctggactgcagctgcagaaagtgaccgtgctgggagtggccacagcccctcagcaggtgctgtctaatggcgtgcccgtgtccaacttcacctacagccccgacaccaaggtgctggacatctgcgtgtcactgctgatgggagagcagtttctggtgtcctggtgctga

SEQ ID NO: 19 - DNA, 2820 bp, artificial
  sp8+hGAAco1-delta-8
atggccagcagactgaccctgctgacactccttctgctgctgctggccggcgatagagccagcagcctactagtgcccagagagctgagcggcagctctcccgtgctggaagaaacacaccctgcccatcagcagggcgcctctagacctggacctagagatgcccaggcccaccccggcagacctagagctgtgcctacccagtgtgacgtgccccccaacagcagattcgactgcgcccctgacaaggccatcacccaggaacagtgcgaggccagaggctgctgctacatccctgccaagcagggactgcagggcgctcagatgggacagccctggtgcttcttcccaccctcctaccccagctacaagctggaaaacctgagcagcagcgagatgggctacaccgccaccctgaccagaaccacccccacattcttcccaaaggacatcctgaccctgcggctggacgtgatgatggaaaccgagaaccggctgcacttcaccatcaaggaccccgccaatcggagatacgaggtgcccctggaaaccccccacgtgcactctagagcccccagccctctgtacagcgtggaattcagcgaggaacccttcggcgtgatcgtgcggagacagctggatggcagagtgctgctgaacaccaccgtggcccctctgttcttcgccgaccagttcctgcagctgagcaccagcctgcccagccagtacatcacaggactggccgagcacctgagccccctgatgctgagcacatcctggacccggatcaccctgtggaacagggatctggcccctacccctggcgccaatctgtacggcagccaccctttctacctggccctggaagatggcggatctgcccacggagtgtttctgctgaactccaacgccatggacgtggtgctgcagcctagccctgccctgtcttggagaagcacaggcggcatcctggatgtgtacatctttctgggccccgagcccaagagcgtggtgcagcagtatctggatgtcgtgggctaccccttcatgcccccttactggggcctgggattccacctgtgcagatggggctactccagcaccgccatcaccagacaggtggtggaaaacatgaccagagcccacttcccactggatgtgcagtggaacgacctggactacatggacagcagacgggacttcaccttcaacaaggacggcttccgggacttccccgccatggtgcaggaactgcatcagggcggcagacggtacatgatgatcgtggatcccgccatcagctcctctggccctgccggctcttacagaccctacgacgagggcctgcggagaggcgtgttcatcaccaacgagacaggccagcccctgatcggcaaagtgtggcctggcagcacagccttccccgacttcaccaatcctaccgccctggcttggtgggaggacatggtggccgagttccacgaccaggtgcccttcgacggcatgtggatcgacatgaacgagcccagcaacttcatccggggcagcgaggatggctgccccaacaacgaactggaaaatcccccttacgtgcccggcgtcgtgggcggaacactgcaggccgctacaatctgtgccagcagccaccagtttctgagcacccactacaacctgcacaacctgtacggcctgaccgaggccattgccagccaccgcgctctcgtgaaagccagaggcacacggcccttcgtgatcagcagaagcacctttgccggccacggcagatacgccggacattggactggcgacgtgtggtcctcttgggagcagctggcctctagcgtgcccgagatcctgcagttcaatctgctgggcgtgccactcgtgggcgccgatgtgtgtggcttcctgggcaacacctccgaggaactgtgtgtgcggtggacacagctgggcgccttctaccctttcatgagaaaccacaacagcctgctgagcctgccccaggaaccctacagctttagcgagcctgcacagcaggccatgcggaaggccctgacactgagatacgctctgctgccccacctgtacaccctgtttcaccaggcccatgtggccggcgagacagtggccagacctctgtttctggaattccccaaggacagcagcacctggaccgtggaccatcagctgctgtggggagaggctctgctgattaccccagtgctgcaggcaggcaaggccgaagtgaccggctactttcccctgggcacttggtacgacctgcagaccgtgcctgtggaagccctgggatctctgcctccacctcctgccgctcctagagagcctgccattcactctgagggccagtgggtcacactgcctgcccccctggataccatcaacgtgcacctgagggccggctacatcataccactgcagggacctggcctgaccaccaccgagtctagacagcagccaatggccctggccgtggccctgaccaaaggcggagaagctaggggcgagctgttctgggacgatggcgagagcctggaagtgctggaaagaggcgcctatacccaagtgatcttcctggcccggaacaacaccatcgtgaacgagctggtgcgcgtgacctctgaaggcgctggactgcagctgcagaaagtgaccgtgctgggagtggccacagcccctcagcaggtgctgtctaatggcgtgcccgtgtccaacttcacctacagccccgacaccaaggtgctggacatctgcgtgtcactgctgatgggagagcagtttctggtgtcctggtgctga

SEQ ID NO: 20 - DNA, 4300 bp, artificial
  construct: sp7+hGAAco1-delta-8
aggctcagaggcacacaggagtttctgggctcaccctgcccccttccaacccctcagttcccatcctccagcagctgtttgtgtgctgcctctgaagtccacactgaacaaacttcagcctactcatgtccctaaaatgggcaaacattgcaagcagcaaacagcaaacacacagccctccctgcctgctgaccttggagctggggcagaggtcagagacctctctgggcccatgccacctccaacatccactcgaccccttggaatttcggtggagaggagcagaggttgtcctggcgtggtttaggtagtgtgagaggggtacccggggatcttgctaccagtggaacagccactaaggattctgcagtgagagcagagggccagctaagtggtactctcccagagactgtctgactcacgccaccccctccaccttggacacaggacgctgtggtttctgagccaggtacaatgactcctttcggtaagtgcagtggaagctgtacactgcccaggcaaagcgtccgggcagcgtaggcgggcgactcagatcccagccagtggacttagcccctgtttgctcctccgataactggggtgaccttggttaatattcaccagcagcctcccccgttgcccctctggatccactgcttaaatacggacgaggacagggccctgtctcctcagcttcaggcaccaccactgacctgggacagtgaatagatcctgagaacttcagggtgagtctatgggacccttgatgttttctttccccttcttttctatggttaagttcatgtcataggaaggggagaagtaacagggtacacatattgaccaaatcagggtaattttgcatttgtaattttaaaaaatgctttcttcttttaatatacttttttgtttatcttatttctaatactttccctaatctctttctttcagggcaataatgatacaatgtatcatgcctctttgcaccattctaaagaataacagtgataatttctgggttaaggcaatagcaatatttctgcatataaatatttctgcatataaattgtaactgatgtaagaggtttcatattgctaatagcagctacaatccagctaccattctgcttttattttctggttgggataaggctggattattctgagtccaagctaggcccttttgctaatcttgttcatacctcttatcttcctcccacagctcctgggcaacctgctggtctctctgctggcccatcactttggcaaagcacgcgtgccaccatggcctttctgtggctgctgagctgttgggccctgctgggcaccaccttcggcctactagtgcccagagagctgagcggcagctctcccgtgctggaagaaacacaccctgcccatcagcagggcgcctctagacctggacctagagatgcccaggcccaccccggcagacctagagctgtgcctacccagtgtgacgtgccccccaacagcagattcgactgcgcccctgacaaggccatcacccaggaacagtgcgaggccagaggctgctgctacatccctgccaagcagggactgcagggcgctcagatgggacagccctggtgcttcttcccaccctcctaccccagctacaagctggaaaacctgagcagcagcgagatgggctacaccgccaccctgaccagaaccacccccacattcttcccaaaggacatcctgaccctgcggctggacgtgatgatggaaaccgagaaccggctgcacttcaccatcaaggaccccgccaatcggagatacgaggtgcccctggaaaccccccacgtgcactctagagcccccagccctctgtacagcgtggaattcagcgaggaacccttcggcgtgatcgtgcggagacagctggatggcagagtgctgctgaacaccaccgtggcccctctgttcttcgccgaccagttcctgcagctgagcaccagcctgcccagccagtacatcacaggactggccgagcacctgagccccctgatgctgagcacatcctggacccggatcaccctgtggaacagggatctggcccctacccctggcgccaatctgtacggcagccaccctttctacctggccctggaagatggcggatctgcccacggagtgtttctgctgaactccaacgccatggacgtggtgctgcagcctagccctgccctgtcttggagaagcacaggcggcatcctggatgtgtacatctttctgggccccgagcccaagagcgtggtgcagcagtatctggatgtcgtgggctaccccttcatgcccccttactggggcctgggattccacctgtgcagatggggctactccagcaccgccatcaccagacaggtggtggaaaacatgaccagagcccacttcccactggatgtgcagtggaacgacctggactacatggacagcagacgggacttcaccttcaacaaggacggcttccgggacttccccgccatggtgcaggaactgcatcagggcggcagacggtacatgatgatcgtggatcccgccatcagctcctctggccctgccggctcttacagaccctacgacgagggcctgcggagaggcgtgttcatcaccaacgagacaggccagcccctgatcggcaaagtgtggcctggcagcacagccttccccgacttcaccaatcctaccgccctggcttggtgggaggacatggtggccgagttccacgaccaggtgcccttcgacggcatgtggatcgacatgaacgagcccagcaacttcatccggggcagcgaggatggctgccccaacaacgaactggaaaatcccccttacgtgcccggcgtcgtgggcggaacactgcaggccgctacaatctgtgccagcagccaccagtttctgagcacccactacaacctgcacaacctgtacggcctgaccgaggccattgccagccaccgcgctctcgtgaaagccagaggcacacggcccttcgtgatcagcagaagcacctttgccggccacggcagatacgccggacattggactggcgacgtgtggtcctcttgggagcagctggcctctagcgtgcccgagatcctgcagttcaatctgctgggcgtgccactcgtgggcgccgatgtgtgtggcttcctgggcaacacctccgaggaactgtgtgtgcggtggacacagctgggcgccttctaccctttcatgagaaaccacaacagcctgctgagcctgccccaggaaccctacagctttagcgagcctgcacagcaggccatgcggaaggccctgacactgagatacgctctgctgccccacctgtacaccctgtttcaccaggcccatgtggccggcgagacagtggccagacctctgtttctggaattccccaaggacagcagcacctggaccgtggaccatcagctgctgtggggagaggctctgctgattaccccagtgctgcaggcaggcaaggccgaagtgaccggctactttcccctgggcacttggtacgacctgcagaccgtgcctgtggaagccctgggatctctgcctccacctcctgccgctcctagagagcctgccattcactctgagggccagtgggtcacactgcctgcccccctggataccatcaacgtgcacctgagggccggctacatcataccactgcagggacctggcctgaccaccaccgagtctagacagcagccaatggccctggccgtggccctgaccaaaggcggagaagctaggggcgagctgttctgggacgatggcgagagcctggaagtgctggaaagaggcgcctatacccaagtgatcttcctggcccggaacaacaccatcgtgaacgagctggtgcgcgtgacctctgaaggcgctggactgcagctgcagaaagtgaccgtgctgggagtggccacagcccctcagcaggtgctgtctaatggcgtgcccgtgtccaacttcacctacagccccgacaccaaggtgctggacatctgcgtgtcactgctgatgggagagcagtttctggtgtcctggtgctgactcgagagatctaccggtgaattcaccgcgggtttaaactgtgccttctagttgccagccatctgttgtttgcccctcccccgtgccttccttgaccctggaaggtgccactcccactgtcctttcctaataaaatgaggaaattgcatcgcattgtctgagtaggtgtcattctattctggggggtggggtgggggctagctctaga

SEQ ID NO: 21 - DNA, 4321 bp, artificial
  construct: sp6+hGAAco1-delta-8
aggctcagaggcacacaggagtttctgggctcaccctgcccccttccaacccctcagttcccatcctccagcagctgtttgtgtgctgcctctgaagtccacactgaacaaacttcagcctactcatgtccctaaaatgggcaaacattgcaagcagcaaacagcaaacacacagccctccctgcctgctgaccttggagctggggcagaggtcagagacctctctgggcccatgccacctccaacatccactcgaccccttggaatttcggtggagaggagcagaggttgtcctggcgtggtttaggtagtgtgagaggggtacccggggatcttgctaccagtggaacagccactaaggattctgcagtgagagcagagggccagctaagtggtactctcccagagactgtctgactcacgccaccccctccaccttggacacaggacgctgtggtttctgagccaggtacaatgactcctttcggtaagtgcagtggaagctgtacactgcccaggcaaagcgtccgggcagcgtaggcgggcgactcagatcccagccagtggacttagcccctgtttgctcctccgataactggggtgaccttggttaatattcaccagcagcctcccccgttgcccctctggatccactgcttaaatacggacgaggacagggccctgtctcctcagcttcaggcaccaccactgacctgggacagtgaatagatcctgagaacttcagggtgagtctatgggacccttgatgttttctttccccttcttttctatggttaagttcatgtcataggaaggggagaagtaacagggtacacatattgaccaaatcagggtaattttgcatttgtaattttaaaaaatgctttcttcttttaatatacttttttgtttatcttatttctaatactttccctaatctctttctttcagggcaataatgatacaatgtatcatgcctctttgcaccattctaaagaataacagtgataatttctgggttaaggcaatagcaatatttctgcatataaatatttctgcatataaattgtaactgatgtaagaggtttcatattgctaatagcagctacaatccagctaccattctgcttttattttctggttgggataaggctggattattctgagtccaagctaggcccttttgctaatcttgttcatacctcttatcttcctcccacagctcctgggcaacctgctggtctctctgctggcccatcactttggcaaagcacgcgtgccaccatgcctccacctagaacaggcagaggcctgctgtggctgggcctggtgctgtctagtgtgtgtgtggccctgggcctactagtgcccagagagctgagcggcagctctcccgtgctggaagaaacacaccctgcccatcagcagggcgcctctagacctggacctagagatgcccaggcccaccccggcagacctagagctgtgcctacccagtgtgacgtgccccccaacagcagattcgactgcgcccctgacaaggccatcacccaggaacagtgcgaggccagaggctgctgctacatccctgccaagcagggactgcagggcgctcagatgggacagccctggtgcttcttcccaccctcctaccccagctacaagctggaaaacctgagcagcagcgagatgggctacaccgccaccctgaccagaaccacccccacattcttcccaaaggacatcctgaccctgcggctggacgtgatgatggaaaccgagaaccggctgcacttcaccatcaaggaccccgccaatcggagatacgaggtgcccctggaaaccccccacgtgcactctagagcccccagccctctgtacagcgtggaattcagcgaggaacccttcggcgtgatcgtgcggagacagctggatggcagagtgctgctgaacaccaccgtggcccctctgttcttcgccgaccagttcctgcagctgagcaccagcctgcccagccagtacatcacaggactggccgagcacctgagccccctgatgctgagcacatcctggacccggatcaccctgtggaacagggatctggcccctacccctggcgccaatctgtacggcagccaccctttctacctggccctggaagatggcggatctgcccacggagtgtttctgctgaactccaacgccatggacgtggtgctgcagcctagccctgccctgtcttggagaagcacaggcggcatcctggatgtgtacatctttctgggccccgagcccaagagcgtggtgcagcagtatctggatgtcgtgggctaccccttcatgcccccttactggggcctgggattccacctgtgcagatggggctactccagcaccgccatcaccagacaggtggtggaaaacatgaccagagcccacttcccactggatgtgcagtggaacgacctggactacatggacagcagacgggacttcaccttcaacaaggacggcttccgggacttccccgccatggtgcaggaactgcatcagggcggcagacggtacatgatgatcgtggatcccgccatcagctcctctggccctgccggctcttacagaccctacgacgagggcctgcggagaggcgtgttcatcaccaacgagacaggccagcccctgatcggcaaagtgtggcctggcagcacagccttccccgacttcaccaatcctaccgccctggcttggtgggaggacatggtggccgagttccacgaccaggtgcccttcgacggcatgtggatcgacatgaacgagcccagcaacttcatccggggcagcgaggatggctgccccaacaacgaactggaaaatcccccttacgtgcccggcgtcgtgggcggaacactgcaggccgctacaatctgtgccagcagccaccagtttctgagcacccactacaacctgcacaacctgtacggcctgaccgaggccattgccagccaccgcgctctcgtgaaagccagaggcacacggcccttcgtgatcagcagaagcacctttgccggccacggcagatacgccggacattggactggcgacgtgtggtcctcttgggagcagctggcctctagcgtgcccgagatcctgcagttcaatctgctgggcgtgccactcgtgggcgccgatgtgtgtggcttcctgggcaacacctccgaggaactgtgtgtgcggtggacacagctgggcgccttctaccctttcatgagaaaccacaacagcctgctgagcctgccccaggaaccctacagctttagcgagcctgcacagcaggccatgcggaaggccctgacactgagatacgctctgctgccccacctgtacaccctgtttcaccaggcccatgtggccggcgagacagtggccagacctctgtttctggaattccccaaggacagcagcacctggaccgtggaccatcagctgctgtggggagaggctctgctgattaccccagtgctgcaggcaggcaaggccgaagtgaccggctactttcccctgggcacttggtacgacctgcagaccgtgcctgtggaagccctgggatctctgcctccacctcctgccgctcctagagagcctgccattcactctgagggccagtgggtcacactgcctgcccccctggataccatcaacgtgcacctgagggccggctacatcataccactgcagggacctggcctgaccaccaccgagtctagacagcagccaatggccctggccgtggccctgaccaaaggcggagaagctaggggcgagctgttctgggacgatggcgagagcctggaagtgctggaaagaggcgcctatacccaagtgatcttcctggcccggaacaacaccatcgtgaacgagctggtgcgcgtgacctctgaaggcgctggactgcagctgcagaaagtgaccgtgctgggagtggccacagcccctcagcaggtgctgtctaatggcgtgcccgtgtccaacttcacctacagccccgacaccaaggtgctggacatctgcgtgtcactgctgatgggagagcagtttctggtgtcctggtgctgactcgagagatctaccggtgaattcaccgcgggtttaaactgtgccttctagttgccagccatctgttgtttgcccctcccccgtgccttccttgaccctggaaggtgccactcccactgtcctttcctaataaaatgaggaaattgcatcgcattgtctgagtaggtgtcattctattctggggggtggggtgggggctagctctaga

SEQ ID NO: 22 - DNA, 4312 bp, artificial
  sp8+hGAAco1-delta-8
aggctcagaggcacacaggagtttctgggctcaccctgcccccttccaacccctcagttcccatcctccagcagctgtttgtgtgctgcctctgaagtccacactgaacaaacttcagcctactcatgtccctaaaatgggcaaacattgcaagcagcaaacagcaaacacacagccctccctgcctgctgaccttggagctggggcagaggtcagagacctctctgggcccatgccacctccaacatccactcgaccccttggaatttcggtggagaggagcagaggttgtcctggcgtggtttaggtagtgtgagaggggtacccggggatcttgctaccagtggaacagccactaaggattctgcagtgagagcagagggccagctaagtggtactctcccagagactgtctgactcacgccaccccctccaccttggacacaggacgctgtggtttctgagccaggtacaatgactcctttcggtaagtgcagtggaagctgtacactgcccaggcaaagcgtccgggcagcgtaggcgggcgactcagatcccagccagtggacttagcccctgtttgctcctccgataactggggtgaccttggttaatattcaccagcagcctcccccgttgcccctctggatccactgcttaaatacggacgaggacagggccctgtctcctcagcttcaggcaccaccactgacctgggacagtgaatagatcctgagaacttcagggtgagtctatgggacccttgatgttttctttccccttcttttctatggttaagttcatgtcataggaaggggagaagtaacagggtacacatattgaccaaatcagggtaattttgcatttgtaattttaaaaaatgctttcttcttttaatatacttttttgtttatcttatttctaatactttccctaatctctttctttcagggcaataatgatacaatgtatcatgcctctttgcaccattctaaagaataacagtgataatttctgggttaaggcaatagcaatatttctgcatataaatatttctgcatataaattgtaactgatgtaagaggtttcatattgctaatagcagctacaatccagctaccattctgcttttattttctggttgggataaggctggattattctgagtccaagctaggcccttttgctaatcttgttcatacctcttatcttcctcccacagctcctgggcaacctgctggtctctctgctggcccatcactttggcaaagcacgcgtgccaccatggccagcagactgaccctgctgacactccttctgctgctgctggccggcgatagagccagcagcctactagtgcccagagagctgagcggcagctctcccgtgctggaagaaacacaccctgcccatcagcagggcgcctctagacctggacctagagatgcccaggcccaccccggcagacctagagctgtgcctacccagtgtgacgtgccccccaacagcagattcgactgcgcccctgacaaggccatcacccaggaacagtgcgaggccagaggctgctgctacatccctgccaagcagggactgcagggcgctcagatgggacagccctggtgcttcttcccaccctcctaccccagctacaagctggaaaacctgagcagcagcgagatgggctacaccgccaccctgaccagaaccacccccacattcttcccaaaggacatcctgaccctgcggctggacgtgatgatggaaaccgagaaccggctgcacttcaccatcaaggaccccgccaatcggagatacgaggtgcccctggaaaccccccacgtgcactctagagcccccagccctctgtacagcgtggaattcagcgaggaacccttcggcgtgatcgtgcggagacagctggatggcagagtgctgctgaacaccaccgtggcccctctgttcttcgccgaccagttcctgcagctgagcaccagcctgcccagccagtacatcacaggactggccgagcacctgagccccctgatgctgagcacatcctggacccggatcaccctgtggaacagggatctggcccctacccctggcgccaatctgtacggcagccaccctttctacctggccctggaagatggcggatctgcccacggagtgtttctgctgaactccaacgccatggacgtggtgctgcagcctagccctgccctgtcttggagaagcacaggcggcatcctggatgtgtacatctttctgggccccgagcccaagagcgtggtgcagcagtatctggatgtcgtgggctaccccttcatgcccccttactggggcctgggattccacctgtgcagatggggctactccagcaccgccatcaccagacaggtggtggaaaacatgaccagagcccacttcccactggatgtgcagtggaacgacctggactacatggacagcagacgggacttcaccttcaacaaggacggcttccgggacttccccgccatggtgcaggaactgcatcagggcggcagacggtacatgatgatcgtggatcccgccatcagctcctctggccctgccggctcttacagaccctacgacgagggcctgcggagaggcgtgttcatcaccaacgagacaggccagcccctgatcggcaaagtgtggcctggcagcacagccttccccgacttcaccaatcctaccgccctggcttggtgggaggacatggtggccgagttccacgaccaggtgcccttcgacggcatgtggatcgacatgaacgagcccagcaacttcatccggggcagcgaggatggctgccccaacaacgaactggaaaatcccccttacgtgcccggcgtcgtgggcggaacactgcaggccgctacaatctgtgccagcagccaccagtttctgagcacccactacaacctgcacaacctgtacggcctgaccgaggccattgccagccaccgcgctctcgtgaaagccagaggcacacggcccttcgtgatcagcagaagcacctttgccggccacggcagatacgccggacattggactggcgacgtgtggtcctcttgggagcagctggcctctagcgtgcccgagatcctgcagttcaatctgctgggcgtgccactcgtgggcgccgatgtgtgtggcttcctgggcaacacctccgaggaactgtgtgtgcggtggacacagctgggcgccttctaccctttcatgagaaaccacaacagcctgctgagcctgccccaggaaccctacagctttagcgagcctgcacagcaggccatgcggaaggccctgacactgagatacgctctgctgccccacctgtacaccctgtttcaccaggcccatgtggccggcgagacagtggccagacctctgtttctggaattccccaaggacagcagcacctggaccgtggaccatcagctgctgtggggagaggctctgctgattaccccagtgctgcaggcaggcaaggccgaagtgaccggctactttcccctgggcacttggtacgacctgcagaccgtgcctgtggaagccctgggatctctgcctccacctcctgccgctcctagagagcctgccattcactctgagggccagtgggtcacactgcctgcccccctggataccatcaacgtgcacctgagggccggctacatcataccactgcagggacctggcctgaccaccaccgagtctagacagcagccaatggccctggccgtggccctgaccaaaggcggagaagctaggggcgagctgttctgggacgatggcgagagcctggaagtgctggaaagaggcgcctatacccaagtgatcttcctggcccggaacaacaccatcgtgaacgagctggtgcgcgtgacctctgaaggcgctggactgcagctgcagaaagtgaccgtgctgggagtggccacagcccctcagcaggtgctgtctaatggcgtgcccgtgtccaacttcacctacagccccgacaccaaggtgctggacatctgcgtgtcactgctgatgggagagcagtttctggtgtcctggtgctgactcgagagatctaccggtgaattcaccgcgggtttaaactgtgccttctagttgccagccatctgttgtttgcccctcccccgtgccttccttgaccctggaaggtgccactcccactgtcctttcctaataaaatgaggaaattgcatcgcattgtctgagtaggtgtcattctattctggggggtggggtgggggctagctctaga

SEQ ID NO: 23 - protein, 16 aa, artificial
  sp3
MLLLSALLLGLAFGYS

SEQ ID NO: 24 - protein, 16 aa, artificial
  sp4
MLLSFALLLGLALGYS

SEQ ID NO: 25 - protein, 16 aa, artificial
  sp5
MLLEHALLLGLAHGYS

SEQ ID NO: 26 - DNA, 54 bp, artificial
  sp7
atggcctttctgtggctgctgagctgttgggccctgctgggcaccaccttcggc

SEQ ID NO: 27 - DNA, 75 bp, artificial
  sp6
atgcctccacctagaacaggcagaggcctgctgtggctgggcctggtgctgtctagtgtgtgtgtggccctgggc

SEQ ID NO: 28 - DNA, 66 bp, artificial
  sp8
atggccagcagactgaccctgctgacactccttctgctgctgctggccggcgatagagccagcagc

SEQ ID NO: 29 - protein, 917 aa, artificial
  hGAA-delta-8
LLVPRELSGSSPVLEETHPAHQQGASRPGPRDAQAHPGRPRAVPTQCDVPPNSRFDCAPDKAITQEQCEARGCCYIPAKQGLQGAQMGQPWCFFPPSYPSYKLENLSSSEMGYTATLTRTTPTFFPKDILTLRLDVMMETENRLHFTIKDPANRRYEVPLETPHVHSRAPSPLYSVEFSEEPFGVIVRRQLDGRVLLNTTVAPLFFADQFLQLSTSLPSQYITGLAEHLSPLMLSTSWTRITLWNRDLAPTPGANLYGSHPFYLALEDGGSAHGVFLLNSNAMDVVLQPSPALSWRSTGGILDVYIFLGPEPKSVVQQYLDVVGYPFMPPYWGLGFHLCRWGYSSTAITRQVVENMTRAHFPLDVQWNDLDYMDSRRDFTFNKDGFRDFPAMVQELHQGGRRYMMIVDPAISSSGPAGSYRPYDEGLRRGVFITNETGQPLIGKVWPGSTAFPDFTNPTALAWWEDMVAEFHDQVPFDGMWIDMNEPSNFIRGSEDGCPNNELENPPYVPGVVGGTLQAATICASSHQFLSTHYNLHNLYGLTEAIASHRALVKARGTRPFVISRSTFAGHGRYAGHWTGDVWSSWEQLASSVPEILQFNLLGVPLVGADVCGFLGNTSEELCVRWTQLGAFYPFMRNHNSLLSLPQEPYSFSEPAQQAMRKALTLRYALLPHLYTLFHQAHVAGETVARPLFLEFPKDSSTWTVDHQLLWGEALLITPVLQAGKAEVTGYFPLGTWYDLQTVPVEALGSLPPPPAAPREPAIHSEGQWVTLPAPLDTINVHLRAGYIIPLQGPGLTTTESRQQPMALAVALTKGGEARGELFWDDGESLEVLERGAYTQVIFLARNNTIVNELVRVTSEGAGLQLQKVTVLGVATAPQQVLSNGVPVSNFTYSPDTKVLDICVSLLMGEQFLVSWC

SEQ ID NO: 30 - protein, 883 aa, artificial
  hGAA-delta-42
AHPGRPRAVPTQCDVPPNSRFDCAPDKAITQEQCEARGCCYIPAKQGLQGAQMGQPWCFFPPSYPSYKLENLSSSEMGYTATLTRTTPTFFPKDILTLRLDVMMETENRLHFTIKDPANRRYEVPLETPHVHSRAPSPLYSVEFSEEPFGVIVRRQLDGRVLLNTTVAPLFFADQFLQLSTSLPSQYITGLAEHLSPLMLSTSWTRITLWNRDLAPTPGANLYGSHPFYLALEDGGSAHGVFLLNSNAMDVVLQPSPALSWRSTGGILDVYIFLGPEPKSVVQQYLDVVGYPFMPPYWGLGFHLCRWGYSSTAITRQVVENMTRAHFPLDVQWNDLDYMDSRRDFTFNKDGFRDFPAMVQELHQGGRRYMMIVDPAISSSGPAGSYRPYDEGLRRGVFITNETGQPLIGKVWPGSTAFPDFTNPTALAWWEDMVAEFHDQVPFDGMWIDMNEPSNFIRGSEDGCPNNELENPPYVPGVVGGTLQAATICASSHQFLSTHYNLHNLYGLTEAIASHRALVKARGTRPFVISRSTFAGHGRYAGHWTGDVWSSWEQLASSVPEILQFNLLGVPLVGADVCGFLGNTSEELCVRWTQLGAFYPFMRNHNSLLSLPQEPYSFSEPAQQAMRKALTLRYALLPHLYTLFHQAHVAGETVARPLFLEFPKDSSTWTVDHQLLWGEALLITPVLQAGKAEVTGYFPLGTWYDLQTVPVEALGSLPPPPAAPREPAIHSEGQWVTLPAPLDTINVHLRAGYIIPLQGPGLTTTESRQQPMALAVALTKGGEARGELFWDDGESLEVLERGAYTQVIFLARNNTIVNELVRVTSEGAGLQLQKVTVLGVATAPQQVLSNGVPVSNFTYSPDTKVLDICVSLLMGEQFLVSWC

SEQ ID NO: 31 - DNA, 2778 bp, hGAAwt w/o sp
gggcacatcctactccatgatttcctgctggttccccgagagctgagtggctcctccccagtcctggaggagactcacccagctcaccagcagggagccagcagaccagggccccgggatgcccaggcacaccccgggcggccgcgagcagtgcccacacagtgcgacgtcccccccaacagccgcttcgattgcgcccctgacaaggccatcacccaggaacagtgcgaggcccgcggctgttgctacatccctgcaaagcaggggctgcagggagcccagatggggcagccctggtgcttcttcccacccagctaccccagctacaagctggagaacctgagctcctctgaaatgggctacacggccaccctgacccgtaccacccccaccttcttccccaaggacatcctgaccctgcggctggacgtgatgatggagactgagaaccgcctccacttcacgatcaaagatccagctaacaggcgctacgaggtgcccttggagaccccgcatgtccacagccgggcaccgtccccactctacagcgtggagttctccgaggagcccttcggggtgatcgtgcgccggcagctggacggccgcgtgctgctgaacacgacggtggcgcccctgttctttgcggaccagttccttcagctgtccacctcgctgccctcgcagtatatcacaggcctcgccgagcacctcagtcccctgatgctcagcaccagctggaccaggatcaccctgtggaaccgggaccttgcgcccacgcccggtgcgaacctctacgggtctcaccctttctacctggcgctggaggacggcgggtcggcacacggggtgttcctgctaaacagcaatgccatggatgtggtcctgcagccgagccctgcccttagctggaggtcgacaggtgggatcctggatgtctacatcttcctgggcccagagcccaagagcgtggtgcagcagtacctggacgttgtgggatacccgttcatgccgccatactggggcctgggcttccacctgtgccgctggggctactcctccaccgctatcacccgccaggtggtggagaacatgaccagggcccacttccccctggacgtccagtggaacgacctggactacatggactcccggagggacttcacgttcaacaaggatggcttccgggacttcccggccatggtgcaggagctgcaccagggcggccggcgctacatgatgatcgtggatcctgccatcagcagctcgggccctgccgggagctacaggccctacgacgagggtctgcggaggggggttttcatcaccaacgagaccggccagccgctgattgggaaggtatggcccgggtccactgccttccccgacttcaccaaccccacagccctggcctggtgggaggacatggtggctgagttccatgaccaggtgcccttcgacggcatgtggattgacatgaacgagccttccaacttcatcaggggctctgaggacggctgccccaacaatgagctggagaacccaccctacgtgcctggggtggttggggggaccctccaggcggccaccatctgtgcctccagccaccagtttctctccacacactacaacctgcacaacctctacggcctgaccgaagccatcgcctcccacagggcgctggtgaaggctcgggggacacgcccatttgtgatctcccgctcgacctttgctggccacggccgatacgccggccactggacgggggacgtgtggagctcctgggagcagctcgcctcctccgtgccagaaatcctgcagtttaacctgctgggggtgcctctggtcggggccgacgtctgcggcttcctgggcaacacctcagaggagctgtgtgtgcgctggacccagctgggggccttctaccccttcatgcggaaccacaacagcctgctcagtctgccccaggagccgtacagcttcagcgagccggcccagcaggccatgaggaaggccctcaccctgcgctacgcactcctcccccacctctacacactgttccaccaggcccacgtcgcgggggagaccgtggcccggcccctcttcctggagttccccaaggactctagcacctggactgtggaccaccagctcctgtggggggaggccctgctcatcaccccagtgctccaggccgggaaggccgaagtgactggctacttccccttgggcacatggtacgacctgcagacggtgccagtagaggcccttggcagcctcccacccccacctgcagctccccgtgagccagccatccacagcgaggggcagtgggtgacgctgccggcccccctggacaccatcaacgtccacctccgggctgggtacatcatccccctgcagggccctggcctcacaaccacagagtcccgccagcagcccatggccctggctgtggccctgaccaagggtggggaggcccgaggggagctgttctgggacgatggagagagcctggaagtgctggagcgaggggcctacacacaggtcatcttcctggccaggaataacacgatcgtgaatgagctggtacgtgtgaccagtgagggagctggcctgcagctgcagaaggtgactgtcctgggcgtggccacggcgccccagcaggtcctctccaacggtgtccctgtctccaacttcacctacagccccgacaccaaggtcctggacatctgtgtctcgctgttgatgggagagcagtttctcgtcagctggtgttag

SEQ ID NO: 32 - DNA, 2754 bp, artificial
  hGAAco1-delta-8 w/o sp
ctactagtgcccagagagctgagcggcagctctcccgtgctggaagaaacacaccctgcccatcagcagggcgcctctagacctggacctagagatgcccaggcccaccccggcagacctagagctgtgcctacccagtgtgacgtgccccccaacagcagattcgactgcgcccctgacaaggccatcacccaggaacagtgcgaggccagaggctgctgctacatccctgccaagcagggactgcagggcgctcagatgggacagccctggtgcttcttcccaccctcctaccccagctacaagctggaaaacctgagcagcagcgagatgggctacaccgccaccctgaccagaaccacccccacattcttcccaaaggacatcctgaccctgcggctggacgtgatgatggaaaccgagaaccggctgcacttcaccatcaaggaccccgccaatcggagatacgaggtgcccctggaaaccccccacgtgcactctagagcccccagccctctgtacagcgtggaattcagcgaggaacccttcggcgtgatcgtgcggagacagctggatggcagagtgctgctgaacaccaccgtggcccctctgttcttcgccgaccagttcctgcagctgagcaccagcctgcccagccagtacatcacaggactggccgagcacctgagccccctgatgctgagcacatcctggacccggatcaccctgtggaacagggatctggcccctacccctggcgccaatctgtacggcagccaccctttctacctggccctggaagatggcggatctgcccacggagtgtttctgctgaactccaacgccatggacgtggtgctgcagcctagccctgccctgtcttggagaagcacaggcggcatcctggatgtgtacatctttctgggccccgagcccaagagcgtggtgcagcagtatctggatgtcgtgggctaccccttcatgcccccttactggggcctgggattccacctgtgcagatggggctactccagcaccgccatcaccagacaggtggtggaaaacatgaccagagcccacttcccactggatgtgcagtggaacgacctggactacatggacagcagacgggacttcaccttcaacaaggacggcttccgggacttccccgccatggtgcaggaactgcatcagggcggcagacggtacatgatgatcgtggatcccgccatcagctcctctggccctgccggctcttacagaccctacgacgagggcctgcggagaggcgtgttcatcaccaacgagacaggccagcccctgatcggcaaagtgtggcctggcagcacagccttccccgacttcaccaatcctaccgccctggcttggtgggaggacatggtggccgagttccacgaccaggtgcccttcgacggcatgtggatcgacatgaacgagcccagcaacttcatccggggcagcgaggatggctgccccaacaacgaactggaaaatcccccttacgtgcccggcgtcgtgggcggaacactgcaggccgctacaatctgtgccagcagccaccagtttctgagcacccactacaacctgcacaacctgtacggcctgaccgaggccattgccagccaccgcgctctcgtgaaagccagaggcacacggcccttcgtgatcagcagaagcacctttgccggccacggcagatacgccggacattggactggcgacgtgtggtcctcttgggagcagctggcctctagcgtgcccgagatcctgcagttcaatctgctgggcgtgccactcgtgggcgccgatgtgtgtggcttcctgggcaacacctccgaggaactgtgtgtgcggtggacacagctgggcgccttctaccctttcatgagaaaccacaacagcctgctgagcctgccccaggaaccctacagctttagcgagcctgcacagcaggccatgcggaaggccctgacactgagatacgctctgctgccccacctgtacaccctgtttcaccaggcccatgtggccggcgagacagtggccagacctctgtttctggaattccccaaggacagcagcacctggaccgtggaccatcagctgctgtggggagaggctctgctgattaccccagtgctgcaggcaggcaaggccgaagtgaccggctactttcccctgggcacttggtacgacctgcagaccgtgcctgtggaagccctgggatctctgcctccacctcctgccgctcctagagagcctgccattcactctgagggccagtgggtcacactgcctgcccccctggataccatcaacgtgcacctgagggccggctacatcataccactgcagggacctggcctgaccaccaccgagtctagacagcagccaatggccctggccgtggccctgaccaaaggcggagaagctaggggcgagctgttctgggacgatggcgagagcctggaagtgctggaaagaggcgcctatacccaagtgatcttcctggcccggaacaacaccatcgtgaacgagctggtgcgcgtgacctctgaaggcgctggactgcagctgcagaaagtgaccgtgctgggagtggccacagcccctcagcaggtgctgtctaatggcgtgcccgtgtccaacttcacctacagccccgacaccaaggtgctggacatctgcgtgtcactgctgatgggagagcagtttctggtgtcctggtgctga

SEQ ID NO: 33 - DNA, 2652 bp, artificial
  hGAAco1-delta-42 w/o sp
gcccaccccggcagacctagagctgtgcctacccagtgtgacgtgccccccaacagcagattcgactgcgcccctgacaaggccatcacccaggaacagtgcgaggccagaggctgctgctacatccctgccaagcagggactgcagggcgctcagatgggacagccctggtgcttcttcccaccctcctaccccagctacaagctggaaaacctgagcagcagcgagatgggctacaccgccaccctgaccagaaccacccccacattcttcccaaaggacatcctgaccctgcggctggacgtgatgatggaaaccgagaaccggctgcacttcaccatcaaggaccccgccaatcggagatacgaggtgcccctggaaaccccccacgtgcactctagagcccccagccctctgtacagcgtggaattcagcgaggaacccttcggcgtgatcgtgcggagacagctggatggcagagtgctgctgaacaccaccgtggcccctctgttcttcgccgaccagttcctgcagctgagcaccagcctgcccagccagtacatcacaggactggccgagcacctgagccccctgatgctgagcacatcctggacccggatcaccctgtggaacagggatctggcccctacccctggcgccaatctgtacggcagccaccctttctacctggccctggaagatggcggatctgcccacggagtgtttctgctgaactccaacgccatggacgtggtgctgcagcctagccctgccctgtcttggagaagcacaggcggcatcctggatgtgtacatctttctgggccccgagcccaagagcgtggtgcagcagtatctggatgtcgtgggctaccccttcatgcccccttactggggcctgggattccacctgtgcagatggggctactccagcaccgccatcaccagacaggtggtggaaaacatgaccagagcccacttcccactggatgtgcagtggaacgacctggactacatggacagcagacgggacttcaccttcaacaaggacggcttccgggacttccccgccatggtgcaggaactgcatcagggcggcagacggtacatgatgatcgtggatcccgccatcagctcctctggccctgccggctcttacagaccctacgacgagggcctgcggagaggcgtgttcatcaccaacgagacaggccagcccctgatcggcaaagtgtggcctggcagcacagccttccccgacttcaccaatcctaccgccctggcttggtgggaggacatggtggccgagttccacgaccaggtgcccttcgacggcatgtggatcgacatgaacgagcccagcaacttcatccggggcagcgaggatggctgccccaacaacgaactggaaaatcccccttacgtgcccggcgtcgtgggcggaacactgcaggccgctacaatctgtgccagcagccaccagtttctgagcacccactacaacctgcacaacctgtacggcctgaccgaggccattgccagccaccgcgctctcgtgaaagccagaggcacacggcccttcgtgatcagcagaagcacctttgccggccacggcagatacgccggacattggactggcgacgtgtggtcctcttgggagcagctggcctctagcgtgcccgagatcctgcagttcaatctgctgggcgtgccactcgtgggcgccgatgtgtgtggcttcctgggcaacacctccgaggaactgtgtgtgcggtggacacagctgggcgccttctaccctttcatgagaaaccacaacagcctgctgagcctgccccaggaaccctacagctttagcgagcctgcacagcaggccatgcggaaggccctgacactgagatacgctctgctgccccacctgtacaccctgtttcaccaggcccatgtggccggcgagacagtggccagacctctgtttctggaattccccaaggacagcagcacctggaccgtggaccatcagctgctgtggggagaggctctgctgattaccccagtgctgcaggcaggcaaggccgaagtgaccggctactttcccctgggcacttggtacgacctgcagaccgtgcctgtggaagccctgggatctctgcctccacctcctgccgctcctagagagcctgccattcactctgagggccagtgggtcacactgcctgcccccctggataccatcaacgtgcacctgagggccggctacatcataccactgcagggacctggcctgaccaccaccgagtctagacagcagccaatggccctggccgtggccctgaccaaaggcggagaagctaggggcgagctgttctgggacgatggcgagagcctggaagtgctggaaagaggcgcctatacccaagtgatcttcctggcccggaacaacaccatcgtgaacgagctggtgcgcgtgacctctgaaggcgctggactgcagctgcagaaagtgaccgtgctgggagtggccacagcccctcagcaggtgctgtctaatggcgtgcccgtgtccaacttcacctacagccccgacaccaaggtgctggacatctgcgtgtcactgctgatgggagagcagtttctggtgtcctggtgctga

SEQ ID NO: 34 - DNA, 2754 bp, artificial
  hGAAco2-delta-8
ctgttggtgcctagagagctgagcggatcatccccagtgctggaggagactcatcctgctcaccaacagggagcttccagaccaggaccgagagacgcccaagcccatcctggtagaccaagagctgtgcctacccaatgcgacgtgccacccaactcccgattcgactgcgcgccagataaggctattacccaagagcagtgtgaagccagaggttgctgctacatcccagcgaagcaaggattgcaaggcgcccaaatgggacaaccttggtgtttcttccccccttcgtacccatcatataaactcgaaaacctgtcctcttcggaaatgggttatactgccaccctcaccagaactactcctactttcttcccgaaagacatcttgaccttgaggctggacgtgatgatggagactgaaaaccggctgcatttcactatcaaagatcctgccaatcggcgatacgaggtccctctggaaacccctcacgtgcactcacgggctccttctccgctttactccgtcgaattctctgaggaacccttcggagtgatcgttagacgccagctggatggtagagtgctgttgaacactactgtggccccacttttcttcgctgaccagtttctgcaactgtccacttccctgccatcccagtacattactggactcgccgaacacctgtcgccactgatgctctcgacctcttggactagaatcactttgtggaacagagacttggcccctactccgggagcaaatctgtacggaagccaccctttttacctggcgctcgaagatggcggatccgctcacggagtgttcctgctgaatagcaacgcaatggacgtggtgctgcaaccttcccctgcactcagttggagaagtaccgggggtattctggacgtgtacatcttcctcggaccagaacccaagagcgtggtgcagcaatatctggacgtggtcggatacccttttatgcctccttactggggactgggattccacctttgccgttggggctactcatccaccgccattaccagacaggtggtggagaatatgaccagagcccacttccctctcgacgtgcagtggaacgatctggactatatggactcccggagagatttcaccttcaacaaggacgggttccgcgattttcccgcgatggttcaagagctccaccagggtggtcgaagatatatgatgatcgtcgacccagccatttcgagcagcggacccgctggatcttatagaccttacgacgaaggccttaggagaggagtgttcatcacaaacgagactggacagcctttgatcggtaaagtgtggcctggatcaaccgcctttcctgactttaccaatcccactgccttggcttggtgggaggacatggtggccgaattccacgaccaagtcccctttgatggaatgtggatcgatatgaacgaaccaagcaattttatcagaggttccgaagacggttgccccaacaacgaactggaaaaccctccttatgtgcccggagtcgtgggcggaacattacaggccgcgactatttgcgccagcagccaccaattcctgtccactcactacaacctccacaacctttatggattaaccgaagctattgcaagtcacagggctctggtgaaggctagagggactaggccctttgtgatctcccgatccacctttgccggacacgggagatacgccggtcactggactggtgacgtgtggagctcatgggaacaactggcctcctccgtgccggaaatcttacagttcaaccttctgggtgtccctcttgtcggagcagacgtgtgtgggtttcttggtaacacctccgaggaactgtgtgtgcgctggactcaactgggtgcattctacccattcatgagaaaccacaactccttgctgtccctgccacaagagccctactcgttcagcgagcctgcacaacaggctatgcggaaggcactgaccctgagatacgccctgcttccacacttatacactctcttccatcaagcgcatgtggcaggagaaaccgttgcaaggcctcttttccttgaattccccaaggattcctcgacttggacggtggatcatcagctgctgtggggagaagctctgctgattactccagtgttgcaagccggaaaagctgaggtgaccggatactttccgctgggaacctggtacgacctccagactgtccctgttgaagcccttggatcactgcctccgcctccggcagctccacgcgaaccagctatacattccgagggacagtgggttacattaccagctcctctggacacaatcaacgtccacttaagagctggctacattatccctctgcaaggaccaggactgactacgaccgagagcagacagcagccaatggcactggctgtggctctgaccaagggaggggaagctagaggagaactcttctgggatgatggggagtcccttgaagtgctggaaagaggcgcttacactcaagtcattttccttgcacggaacaacaccattgtgaacgaattggtgcgagtgaccagcgaaggagctggacttcaactgcagaaggtcactgtgctcggagtggctaccgctcctcagcaagtgctgtcgaatggagtccccgtgtcaaactttacctactcccctgacactaaggtgctcgacatttgcgtgtccctcctgatgggagagcagttccttgtgtcctggtgttga

SEQ ID NO: 35 - DNA, 2652 bp, artificial
  hGAAco2-delta-42
gcccatcctggtagaccaagagctgtgcctacccaatgcgacgtgccacccaactcccgattcgactgcgcgccagataaggctattacccaagagcagtgtgaagccagaggttgctgctacatcccagcgaagcaaggattgcaaggcgcccaaatgggacaaccttggtgtttcttccccccttcgtacccatcatataaactcgaaaacctgtcctcttcggaaatgggttatactgccaccctcaccagaactactcctactttcttcccgaaagacatcttgaccttgaggctggacgtgatgatggagactgaaaaccggctgcatttcactatcaaagatcctgccaatcggcgatacgaggtccctctggaaacccctcacgtgcactcacgggctccttctccgctttactccgtcgaattctctgaggaacccttcggagtgatcgttagacgccagctggatggtagagtgctgttgaacactactgtggccccacttttcttcgctgaccagtttctgcaactgtccacttccctgccatcccagtacattactggactcgccgaacacctgtcgccactgatgctctcgacctcttggactagaatcactttgtggaacagagacttggcccctactccgggagcaaatctgtacggaagccaccctttttacctggcgctcgaagatggcggatccgctcacggagtgttcctgctgaatagcaacgcaatggacgtggtgctgcaaccttcccctgcactcagttggagaagtaccgggggtattctggacgtgtacatcttcctcggaccagaacccaagagcgtggtgcagcaatatctggacgtggtcggatacccttttatgcctccttactggggactgggattccacctttgccgttggggctactcatccaccgccattaccagacaggtggtggagaatatgaccagagcccacttccctctcgacgtgcagtggaacgatctggactatatggactcccggagagatttcaccttcaacaaggacgggttccgcgattttcccgcgatggttcaagagctccaccagggtggtcgaagatatatgatgatcgtcgacccagccatttcgagcagcggacccgctggatcttatagaccttacgacgaaggccttaggagaggagtgttcatcacaaacgagactggacagcctttgatcggtaaagtgtggcctggatcaaccgcctttcctgactttaccaatcccactgccttggcttggtgggaggacatggtggccgaattccacgaccaagtcccctttgatggaatgtggatcgatatgaacgaaccaagcaattttatcagaggttccgaagacggttgccccaacaacgaactggaaaaccctccttatgtgcccggagtcgtgggcggaacattacaggccgcgactatttgcgccagcagccaccaattcctgtccactcactacaacctccacaacctttatggattaaccgaagctattgcaagtcacagggctctggtgaaggctagagggactaggccctttgtgatctcccgatccacctttgccggacacgggagatacgccggtcactggactggtgacgtgtggagctcatgggaacaactggcctcctccgtgccggaaatcttacagttcaaccttctgggtgtccctcttgtcggagcagacgtgtgtgggtttcttggtaacacctccgaggaactgtgtgtgcgctggactcaactgggtgcattctacccattcatgagaaaccacaactccttgctgtccctgccacaagagccctactcgttcagcgagcctgcacaacaggctatgcggaaggcactgaccctgagatacgccctgcttccacacttatacactctcttccatcaagcgcatgtggcaggagaaaccgttgcaaggcctcttttccttgaattccccaaggattcctcgacttggacggtggatcatcagctgctgtggggagaagctctgctgattactccagtgttgcaagccggaaaagctgaggtgaccggatactttccgctgggaacctggtacgacctccagactgtccctgttgaagcccttggatcactgcctccgcctccggcagctccacgcgaaccagctatacattccgagggacagtgggttacattaccagctcctctggacacaatcaacgtccacttaagagctggctacattatccctctgcaaggaccaggactgactacgaccgagagcagacagcagccaatggcactggctgtggctctgaccaagggaggggaagctagaggagaactcttctgggatgatggggagtcccttgaagtgctggaaagaggcgcttacactcaagtcattttccttgcacggaacaacaccattgtgaacgaattggtgcgagtgaccagcgaaggagctggacttcaactgcagaaggtcactgtgctcggagtggctaccgctcctcagcaagtgctgtcgaatggagtccccgtgtcaaactttacctactcccctgacactaaggtgctcgacatttgcgtgtccctcctgatgggagagcagttccttgtgtcctggtgttga

SEQ ID NO: 36 - protein, 925 aa, artificial
  variant hGAAwt w/o sp
GHILLHDFLLVPRELSGSSPVLEETHPAHQQGASRPGPRDAQAHPGRPRAVPTQCDVPPNSRFDCAPDKAITQEQCEARGCCYIPAKQGLQGAQMGQPWCFFPPSYPSYKLENLSSSEMGYTATLTRTTPTFFPKDILTLRLDVMMETENRLHFTIKDPANRRYEVPLETPRVHSRAPSPLYSVEFSEEPFGVIVHRQLDGRVLLNTTVAPLFFADQFLQLSTSLPSQYITGLAEHLSPLMLSTSWTRITLWNRDLAPTPGANLYGSHPFYLALEDGGSAHGVFLLNSNAMDVVLQPSPALSWRSTGGILDVYIFLGPEPKSVVQQYLDVVGYPFMPPYWGLGFHLCRWGYSSTAITRQVVENMTRAHFPLDVQWNDLDYMDSRRDFTFNKDGFRDFPAMVQELHQGGRRYMMIVDPAISSSGPAGSYRPYDEGLRRGVFITNETGQPLIGKVWPGSTAFPDFTNPTALAWWEDMVAEFHDQVPFDGMWIDMNEPSNFIRGSEDGCPNNELENPPYVPGVVGGTLQAATICASSHQFLSTHYNLHNLYGLTEAIASHRALVKARGTRPFVISRSTFAGHGRYAGHWTGDVWSSWEQLASSVPEILQFNLLGVPLVGADVCGFLGNTSEELCVRWTQLGAFYPFMRNHNSLLSLPQEPYSFSEPAQQAMRKALTLRYALLPHLYTLFHQAHVAGETVARPLFLEFPKDSSTWTVDHQLLWGEALLITPVLQAGKAEVTGYFPLGTWYDLQTVPIEALGSLPPPPAAPREPAIHSEGQWVTLPAPLDTINVHLRAGYIIPLQGPGLTTTESRQQPMALAVALTKGGEARGELFWDDGESLEVLERGAYTQVIFLARNNTIVNELVRVTSEGAGLQLQKVTVLGVATAPQQVLSNGVPVSNFTYSPDTKVLDICVSLLMGEQFLVSWC

SEQ ID NO: 37 - protein, 952 aa, homo sapiens
MGVRHPPCSHRLLAVCALVSLATAALLGHILLHDFLLVPRELSGSSPVLEETHPAHQQGASRPGPRDAQAHPGRPRAVPTQCDVPPNSRFDCAPDKAITQEQCEARGCCYIPAKQGLQGAQMGQPWCFFPPSYPSYKLENLSSSEMGYTATLTRTTPTFFPKDILTLRLDVMMETENRLHFTIKDPANRRYEVPLETPRVHSRAPSPLYSVEFSEEPFGVIVHRQLDGRVLLNTTVAPLFFADQFLQLSTSLPSQYITGLAEHLSPLMLSTSWTRITLWNRDLAPTPGANLYGSHPFYLALEDGGSAHGVFLLNSNAMDVVLQPSPALSWRSTGGILDVYIFLGPEPKSVVQQYLDVVGYPFMPPYWGLGFHLCRWGYSSTAITRQVVENMTRAHFPLDVQWNDLDYMDSRRDFTFNKDGFRDFPAMVQELHQGGRRYMMIVDPAISSSGPAGSYRPYDEGLRRGVFITNETGQPLIGKVWPGSTAFPDFTNPTALAWWEDMVAEFHDQVPFDGMWIDMNEPSNFIRGSEDGCPNNELENPPYVPGVVGGTLQAATICASSHQFLSTHYNLHNLYGLTEAIASHRALVKARGTRPFVISRSTFAGHGRYAGHWTGDVWSSWEQLASSVPEILQFNLLGVPLVGADVCGFLGNTSEELCVRWTQLGAFYPFMRNHNSLLSLPQEPYSFSEPAQQAMRKALTLRYALLPHLYTLFHQAHVAGETVARPLFLEFPKDSSTWTVDHQLLWGEALLITPVLQAGKAEVTGYFPLGTWYDLQTVPIEALGSLPPPPAAPREPAIHSEGQWVTLPAPLDTINVHLRAGYIIPLQGPGLTTTESRQQPMALAVALTKGGEARGELFWDDGESLEVLERGAYTQVIFLARNNTIVNELVRVTSEGAGLQLQKVTVLGVATAPQQVLSNGVPVSNFTYSPDTKVLDICVSLLMGEQFLVSWC

SEQ ID NO: 38 - protein, 952 aa, homo sapiens [sequence omitted]

SEQ ID NO: 39 - protein, 957 aa, homo sapiens [sequence omitted]

SEQ ID NO: 40 - protein, 952 aa, homo sapiens [sequence omitted]

SEQ ID NO: 41 - protein, 896 aa, artificial
  hGAA-delta-29
QQGASRPGPRDAQAHPGRPRAVPTQCDVPPNSRFDCAPDKAITQEQCEARGCCYIPAKQGLQGAQMGQPWCFFPPSYPSYKLENLSSSEMGYTATLTRTTPTFFPKDILTLRLDVMMETENRLHFTIKDPANRRYEVPLETPHVHSRAPSPLYSVEFSEEPFGVIVRRQLDGRVLLNTTVAPLFFADQFLQLSTSLPSQYITGLAEHLSPLMLSTSWTRITLWNRDLAPTPGANLYGSHPFYLALEDGGSAHGVFLLNSNAMDVVLQPSPALSWRSTGGILDVYIFLGPEPKSVVQQYLDVVGYPFMPPYWGLGFHLCRWGYSSTAITRQVVENMTRAHFPLDVQWNDLDYMDSRRDFTFNKDGFRDFPAMVQELHQGGRRYMMIVDPAISSSGPAGSYRPYDEGLRRGVFITNETGQPLIGKVWPGSTAFPDFTNPTALAWWEDMVAEFHDQVPFDGMWIDMNEPSNFIRGSEDGCPNNELENPPYVPGVVGGTLQAATICASSHQFLSTHYNLHNLYGLTEAIASHRALVKARGTRPFVISRSTFAGHGRYAGHWTGDVWSSWEQLASSVPEILQFNLLGVPLVGADVCGFLGNTSEELCVRWTQLGAFYPFMRNHNSLLSLPQEPYSFSEPAQQAMRKALTLRYALLPHLYTLFHQAHVAGETVARPLFLEFPKDSSTWTVDHQLLWGEALLITPVLQAGKAEVTGYFPLGTWYDLQTVPVEALGSLPPPPAAPREPAIHSEGQWVTLPAPLDTINVHLRAGYIIPLQGPGLTTTESRQQPMALAVALTKGGEARGELFWDDGESLEVLERGAYTQVIFLARNNTIVNELVRVTSEGAGLQLQKVTVLGVATAPQQVLSNGVPVSNFTYSPDTKVLDICVSLLMGEQFLVSWC

SEQ ID NO: 42 - protein, 882 aa, artificial
  hGAA-delta-43
HPGRPRAVPTQCDVPPNSRFDCAPDKAITQEQCEARGCCYIPAKQGLQGAQMGQPWCFFPPSYPSYKLENLSSSEMGYTATLTRTTPTFFPKDILTLRLDVMMETENRLHFTIKDPANRRYEVPLETPHVHSRAPSPLYSVEFSEEPFGVIVRRQLDGRVLLNTTVAPLFFADQFLQLSTSLPSQYITGLAEHLSPLMLSTSWTRITLWNRDLAPTPGANLYGSHPFYLALEDGGSAHGVFLLNSNAMDVVLQPSPALSWRSTGGILDVYIFLGPEPKSVVQQYLDVVGYPFMPPYWGLGFHLCRWGYSSTAITRQVVENMTRAHFPLDVQWNDLDYMDSRRDFTFNKDGFRDFPAMVQELHQGGRRYMMIVDPAISSSGPAGSYRPYDEGLRRGVFITNETGQPLIGKVWPGSTAFPDFTNPTALAWWEDMVAEFHDQVPFDGMWIDMNEPSNFIRGSEDGCPNNELENPPYVPGVVGGTLQAATICASSHQFLSTHYNLHNLYGLTEAIASHRALVKARGTRPFVISRSTFAGHGRYAGHWTGDVWSSWEQLASSVPEILQFNLLGVPLVGADVCGFLGNTSEELCVRWTQLGAFYPFMRNHNSLLSLPQEPYSFSEPAQQAMRKALTLRYALLPHLYTLFHQAHVAGETVARPLFLEFPKDSSTWTVDHQLLWGEALLITPVLQAGKAEVTGYFPLGTWYDLQTVPVEALGSLPPPPAAPREPAIHSEGQWVTLPAPLDTINVHLRAGYIIPLQGPGLTTTESRQQPMALAVALTKGGEARGELFWDDGESLEVLERGAYTQVIFLARNNTIVNELVRVTSEGAGLQLQKVTVLGVATAPQQVLSNGVPVSNFTYSPDTKVLDICVSLLMGEQFLVSWC

SEQ ID NO: 43 - protein, 878 aa, artificial
  hGAA-delta-47
PRAVPTQCDVPPNSRFDCAPDKAITQEQCEARGCCYIPAKQGLQGAQMGQPWCFFPPSYPSYKLENLSSSEMGYTATLTRTTPTFFPKDILTLRLDVMMETENRLHFTIKDPANRRYEVPLETPHVHSRAPSPLYSVEFSEEPFGVIVRRQLDGRVLLNTTVAPLFFADQFLQLSTSLPSQYITGLAEHLSPLMLSTSWTRITLWNRDLAPTPGANLYGSHPFYLALEDGGSAHGVFLLNSNAMDVVLQPSPALSWRSTGGILDVYIFLGPEPKSVVQQYLDVVGYPFMPPYWGLGFHLCRWGYSSTAITRQVVENMTRAHFPLDVQWNDLDYMDSRRDFTFNKDGFRDFPAMVQELHQGGRRYMMIVDPAISSSGPAGSYRPYDEGLRRGVFITNETGQPLIGKVWPGSTAFPDFTNPTALAWWEDMVAEFHDQVPFDGMWIDMNEPSNFIRGSEDGCPNNELENPPYVPGVVGGTLQAATICASSHQFLSTHYNLHNLYGLTEAIASHRALVKARGTRPFVISRSTFAGHGRYAGHWTGDVWSSWEQLASSVPEILQFNLLGVPLVGADVCGFLGNTSEELCVRWTQLGAFYPFMRNHNSLLSLPQEPYSFSEPAQQAMRKALTLRYALLPHLYTLFHQAHVAGETVARPLFLEFPKDSSTWTVDHQLLWGEALLITPVLQAGKAEVTGYFPLGTWYDLQTVPVEALGSLPPPPAAPREPAIHSEGQWVTLPAPLDTINVHLRAGYIIPLQGPGLTTTESRQQPMALAVALTKGGEARGELFWDDGESLEVLERGAYTQVIFLARNNTIVNELVRVTSEGAGLQLQKVTVLGVATAPQQVLSNGVPVSNFTYSPDTKVLDICVSLLMGEQFLVSWC

SEQ ID NO: 44 - DNA, 2754 bp, artificial
  hGAAwt-delta-8
ctgctggttccccgagagctgagtggctcctccccagtcctggaggagactcacccagctcaccagcagggagccagcagaccagggccccgggatgcccaggcacaccccgggcggccgcgagcagtgcccacacagtgcgacgtcccccccaacagccgcttcgattgcgcccctgacaaggccatcacccaggaacagtgcgaggcccgcggctgttgctacatccctgcaaagcaggggctgcagggagcccagatggggcagccctggtgcttcttcccacccagctaccccagctacaagctggagaacctgagctcctctgaaatgggctacacggccaccctgacccgtaccacccccaccttcttccccaaggacatcctgaccctgcggctggacgtgatgatggagactgagaaccgcctccacttcacgatcaaagatccagctaacaggcgctacgaggtgcccttggagaccccgcatgtccacagccgggcaccgtccccactctacagcgtggagttctccgaggagcccttcggggtgatcgtgcgccggcagctggacggccgcgtgctgctgaacacgacggtggcgcccctgttctttgcggaccagttccttcagctgtccacctcgctgccctcgcagtatatcacaggcctcgccgagcacctcagtcccctgatgctcagcaccagctggaccaggatcaccctgtggaaccgggaccttgcgcccacgcccggtgcgaacctctacgggtctcaccctttctacctggcgctggaggacggcgggtcggcacacggggtgttcctgctaaacagcaatgccatggatgtggtcctgcagccgagccctgcccttagctggaggtcgacaggtgggatcctggatgtctacatcttcctgggcccagagcccaagagcgtggtgcagcagtacctggacgttgtgggatacccgttcatgccgccatactggggcctgggcttccacctgtgccgctggggctactcctccaccgctatcacccgccaggtggtggagaacatgaccagggcccacttccccctggacgtccagtggaacgacctggactacatggactcccggagggacttcacgttcaacaaggatggcttccgggacttcccggccatggtgcaggagctgcaccagggcggccggcgctacatgatgatcgtggatcctgccatcagcagctcgggccctgccgggagctacaggccctacgacgagggtctgcggaggggggttttcatcaccaacgagaccggccagccgctgattgggaaggtatggcccgggtccactgccttccccgacttcaccaaccccacagccctggcctggtgggaggacatggtggctgagttccatgaccaggtgcccttcgacggcatgtggattgacatgaacgagccttccaacttcatcaggggctctgaggacggctgccccaacaatgagctggagaacccaccctacgtgcctggggtggttggggggaccctccaggcggccaccatctgtgcctccagccaccagtttctctccacacactacaacctgcacaacctctacggcctgaccgaagccatcgcctcccacagggcgctggtgaaggctcgggggacacgcccatttgtgatctcccgctcgacctttgctggccacggccgatacgccggccactggacgggggacgtgtggagctcctgggagcagctcgcctcctccgtgccagaaatcctgcagtttaacctgctgggggtgcctctggtcggggccgacgtctgcggcttcctgggcaacacctcagaggagctgtgtgtgcgctggacccagctgggggccttctaccccttcatgcggaaccacaacagcctgctcagtctgccccaggagccgtacagcttcagcgagccggcccagcaggccatgaggaaggccctcaccctgcgctacgcactcctcccccacctctacacactgttccaccaggcccacgtcgcgggggagaccgtggcccggcccctcttcctggagttccccaaggactctagcacctggactgtggaccaccagctcctgtggggggaggccctgctcatcaccccagtgctccaggccgggaaggccgaagtgactggctacttccccttgggcacatggtacgacctgcagacggtgccagtagaggcccttggcagcctcccacccccacctgcagctccccgtgagccagccatccacagcgaggggcagtgggtgacgctgccggcccccctggacaccatcaacgtccacctccgggctgggtacatcatccccctgcagggccctggcctcacaaccacagagtcccgccagcagcccatggccctggctgtggccctgaccaagggtggggaggcccgaggggagctgttctgggacgatggagagagcctggaagtgctggagcgaggggcctacacacaggtcatcttcctggccaggaataacacgatcgtgaatgagctggtacgtgtgaccagtgagggagctggcctgcagctgcagaaggtgactgtcctgggcgtggccacggcgccccagcaggtcctctccaacggtgtccctgtctccaacttcacctacagccccgacaccaaggtcctggacatctgtgtctcgctgttgatgggagagcagtttctcgtcagctggtgttag

SEQ ID NO: 45 - DNA, 2691 bp, artificial
  hGAAwt-delta-29
cagcagggagccagcagaccagggccccgggatgcccaggcacaccccgggcggccgcgagcagtgcccacacagtgcgacgtcccccccaacagccgcttcgattgcgcccctgacaaggccatcacccaggaacagtgcgaggcccgcggctgttgctacatccctgcaaagcaggggctgcagggagcccagatggggcagccctggtgcttcttcccacccagctaccccagctacaagctggagaacctgagctcctctgaaatgggctacacggccaccctgacccgtaccacccccaccttcttccccaaggacatcctgaccctgcggctggacgtgatgatggagactgagaaccgcctccacttcacgatcaaagatccagctaacaggcgctacgaggtgcccttggagaccccgcatgtccacagccgggcaccgtccccactctacagcgtggagttctccgaggagcccttcggggtgatcgtgcgccggcagctggacggccgcgtgctgctgaacacgacggtggcgcccctgttctttgcggaccagttccttcagctgtccacctcgctgccctcgcagtatatcacaggcctcgccgagcacctcagtcccctgatgctcagcaccagctggaccaggatcaccctgtggaaccgggaccttgcgcccacgcccggtgcgaacctctacgggtctcaccctttctacctggcgctggaggacggcgggtcggcacacggggtgttcctgctaaacagcaatgccatggatgtggtcctgcagccgagccctgcccttagctggaggtcgacaggtgggatcctggatgtctacatcttcctgggcccagagcccaagagcgtggtgcagcagtacctggacgttgtgggatacccgttcatgccgccatactggggcctgggcttccacctgtgccgctggggctactcctccaccgctatcacccgccaggtggtggagaacatgaccagggcccacttccccctggacgtccagtggaacgacctggactacatggactcccggagggacttcacgttcaacaaggatggcttccgggacttcccggccatggtgcaggagctgcaccagggcggccggcgctacatgatgatcgtggatcctgccatcagcagctcgggccctgccgggagctacaggccctacgacgagggtctgcggaggggggttttcatcaccaacgagaccggccagccgctgattgggaaggtatggcccgggtccactgccttccccgacttcaccaaccccacagccctggcctggtgggaggacatggtggctgagttccatgaccaggtgcccttcgacggcatgtggattgacatgaacgagccttccaacttcatcaggggctctgaggacggctgccccaacaatgagctggagaacccaccctacgtgcctggggtggttggggggaccctccaggcggccaccatctgtgcctccagccaccagtttctctccacacactacaacctgcacaacctctacggcctgaccgaagccatcgcctcccacagggcgctggtgaaggctcgggggacacgcccatttgtgatctcccgctcgacctttgctggccacggccgatacgccggccactggacgggggacgtgtggagctcctgggagcagctcgcctcctccgtgccagaaatcctgcagtttaacctgctgggggtgcctctggtcggggccgacgtctgcggcttcctgggcaacacctcagaggagctgtgtgtgcgctggacccagctgggggccttctaccccttcatgcggaaccacaacagcctgctcagtctgccccaggagccgtacagcttcagcgagccggcccagcaggccatgaggaaggccctcaccctgcgctacgcactcctcccccacctctacacactgttccaccaggcccacgtcgcgggggagaccgtggcccggcccctcttcctggagttccccaaggactctagcacctggactgtggaccaccagctcctgtggggggaggccctgctcatcaccccagtgctccaggccgggaaggccgaagtgactggctacttccccttgggcacatggtacgacctgcagacggtgccagtagaggcccttggcagcctcccacccccacctgcagctccccgtgagccagccatccacagcgaggggcagtgggtgacgctgccggcccccctggacaccatcaacgtccacctccgggctgggtacatcatccccctgcagggccctggcctcacaaccacagagtcccgccagcagcccatggccctggctgtggccctgaccaagggtggggaggcccgaggggagctgttctgggacgatggagagagcctggaagtgctggagcgaggggcctacacacaggtcatcttcctggccaggaataacacgatcgtgaatgagctggtacgtgtgaccagtgagggagctggcctgcagctgcagaaggtgactgtcctgggcgtggccacggcgccccagcaggtcctctccaacggtgtccctgtctccaacttcacctacagccccgacaccaaggtcctggacatctgtgtctcgctgttgatgggagagcagtttctcgtcagctggtgttag

SEQ ID NO: 46 - DNA, 2691 bp, artificial
  hGAAco1-delta-29
cagcagggcgcctctagacctggacctagagatgcccaggcccaccccggcagacctagagctgtgcctacccagtgtgacgtgccccccaacagcagattcgactgcgcccctgacaaggccatcacccaggaacagtgcgaggccagaggctgctgctacatccctgccaagcagggactgcagggcgctcagatgggacagccctggtgcttcttcccaccctcctaccccagctacaagctggaaaacctgagcagcagcgagatgggctacaccgccaccctgaccagaaccacccccacattcttcccaaaggacatcctgaccctgcggctggacgtgatgatggaaaccgagaaccggctgcacttcaccatcaaggaccccgccaatcggagatacgaggtgcccctggaaaccccccacgtgcactctagagcccccagccctctgtacagcgtggaattcagcgaggaacccttcggcgtgatcgtgcggagacagctggatggcagagtgctgctgaacaccaccgtggcccctctgttcttcgccgaccagttcctgcagctgagcaccagcctgcccagccagtacatcacaggactggccgagcacctgagccccctgatgctgagcacatcctggacccggatcaccctgtggaacagggatctggcccctacccctggcgccaatctgtacggcagccaccctttctacctggccctggaagatggcggatctgcccacggagtgtttctgctgaactccaacgccatggacgtggtgctgcagcctagccctgccctgtcttggagaagcacaggcggcatcctggatgtgtacatctttctgggccccgagcccaagagcgtggtgcagcagtatctggatgtcgtgggctaccccttcatgcccccttactggggcctgggattccacctgtgcagatggggctactccagcaccgccatcaccagacaggtggtggaaaacatgaccagagcccacttcccactggatgtgcagtggaacgacctggactacatggacagcagacgggacttcaccttcaacaaggacggcttccgggacttccccgccatggtgcaggaactgcatcagggcggcagacggtacatgatgatcgtggatcccgccatcagctcctctggccctgccggctcttacagaccctacgacgagggcctgcggagaggcgtgttcatcaccaacgagacaggccagcccctgatcggcaaagtgtggcctggcagcacagccttccccgacttcaccaatcctaccgccctggcttggtgggaggacatggtggccgagttccacgaccaggtgcccttcgacggcatgtggatcgacatgaacgagcccagcaacttcatccggggcagcgaggatggctgccccaacaacgaactggaaaatcccccttacgtgcccggcgtcgtgggcggaacactgcaggccgctacaatctgtgccagcagccaccagtttctgagcacccactacaacctgcacaacctgtacggcctgaccgaggccattgccagccaccgcgctctcgtgaaagccagaggcacacggcccttcgtgatcagcagaagcacctttgccggccacggcagatacgccggacattggactggcgacgtgtggtcctcttgggagcagctggcctctagcgtgcccgagatcctgcagttcaatctgctgggcgtgccactcgtgggcgccgatgtgtgtggcttcctgggcaacacctccgaggaactgtgtgtgcggtggacacagctgggcgccttctaccctttcatgagaaaccacaacagcctgctgagcctgccccaggaaccctacagctttagcgagcctgcacagcaggccatgcggaaggccctgacactgagatacgctctgctgccccacctgtacaccctgtttcaccaggcccatgtggccggcgagacagtggccagacctctgtttctggaattccccaaggacagcagcacctggaccgtggaccatcagctgctgtggggagaggctctgctgattaccccagtgctgcaggcaggcaaggccgaagtgaccggctactttcccctgggcacttggtacgacctgcagaccgtgcctgtggaagccctgggatctctgcctccacctcctgccgctcctagagagcctgccattcactctgagggccagtgggtcacactgcctgcccccctggataccatcaacgtgcacctgagggccggctacatcataccactgcagggacctggcctgaccaccaccgagtctagacagcagccaatggccctggccgtggccctgaccaaaggcggagaagctaggggcgagctgttctgggacgatggcgagagcctggaagtgctggaaagaggcgcctatacccaagtgatcttcctggcccggaacaacaccatcgtgaacgagctggtgcgcgtgacctctgaaggcgctggactgcagctgcagaaagtgaccgtgctgggagtggccacagcccctcagcaggtgctgtctaatggcgtgcccgtgtccaacttcacctacagccccgacaccaaggtgctggacatctgcgtgtcactgctgatgggagagcagtttctggtgtcctggtgctga

SEQ ID NO: 47 - DNA, 2691 bp, artificial
  hGAAco2-delta-29
caacagggagcttccagaccaggaccgagagacgcccaagcccatcctggtagaccaagagctgtgcctacccaatgcgacgtgccacccaactcccgattcgactgcgcgccagataaggctattacccaagagcagtgtgaagccagaggttgctgctacatcccagcgaagcaaggattgcaaggcgcccaaatgggacaaccttggtgtttcttccccccttcgtacccatcatataaactcgaaaacctgtcctcttcggaaatgggttatactgccaccctcaccagaactactcctactttcttcccgaaagacatcttgaccttgaggctggacgtgatgatggagactgaaaaccggctgcatttcactatcaaagatcctgccaatcggcgatacgaggtccctctggaaacccctcacgtgcactcacgggctccttctccgctttactccgtcgaattctctgaggaacccttcggagtgatcgttagacgccagctggatggtagagtgctgttgaacactactgtggccccacttttcttcgctgaccagtttctgcaactgtccacttccctgccatcccagtacattactggactcgccgaacacctgtcgccactgatgctctcgacctcttggactagaatcactttgtggaacagagacttggcccctactccgggagcaaatctgtacggaagccaccctttttacctggcgctcgaagatggcggatccgctcacggagtgttcctgctgaatagcaacgcaatggacgtggtgctgcaaccttcccctgcactcagttggagaagtaccgggggtattctggacgtgtacatcttcctcggaccagaacccaagagcgtggtgcagcaatatctggacgtggtcggatacccttttatgcctccttactggggactgggattccacctttgccgttggggctactcatccaccgccattaccagacaggtggtggagaatatgaccagagcccacttccctctcgacgtgcagtggaacgatctggactatatggactcccggagagatttcaccttcaacaaggacgggttccgcgattttcccgcgatggttcaagagctccaccagggtggtcgaagatatatgatgatcgtcgacccagccatttcgagcagcggacccgctggatcttatagaccttacgacgaaggccttaggagaggagtgttcatcacaaacgagactggacagcctttgatcggtaaagtgtggcctggatcaaccgcctttcctgactttaccaatcccactgccttggcttggtgggaggacatggtggccgaattccacgaccaagtcccctttgatggaatgtggatcgatatgaacgaaccaagcaattttatcagaggttccgaagacggttgccccaacaacgaactggaaaaccctccttatgtgcccggagtcgtgggcggaacattacaggccgcgactatttgcgccagcagccaccaattcctgtccactcactacaacctccacaacctttatggattaaccgaagctattgcaagtcacagggctctggtgaaggctagagggactaggccctttgtgatctcccgatccacctttgccggacacgggagatacgccggtcactggactggtgacgtgtggagctcatgggaacaactggcctcctccgtgccggaaatcttacagttcaaccttctgggtgtccctcttgtcggagcagacgtgtgtgggtttcttggtaacacctccgaggaactgtgtgtgcgctggactcaactgggtgcattctacccattcatgagaaaccacaactccttgctgtccctgccacaagagccctactcgttcagcgagcctgcacaacaggctatgcggaaggcactgaccctgagatacgccctgcttccacacttatacactctcttccatcaagcgcatgtggcaggagaaaccgttgcaaggcctcttttccttgaattccccaaggattcctcgacttggacggtggatcatcagctgctgtggggagaagctctgctgattactccagtgttgcaagccggaaaagctgaggtgaccggatactttccgctgggaacctggtacgacctccagactgtccctgttgaagcccttggatcactgcctccgcctccggcagctccacgcgaaccagctatacattccgagggacagtgggttacattaccagctcctctggacacaatcaacgtccacttaagagctggctacattatccctctgcaaggaccaggactgactacgaccgagagcagacagcagccaatggcactggctgtggctctgaccaagggaggggaagctagaggagaactcttctgggatgatggggagtcccttgaagtgctggaaagaggcgcttacactcaagtcattttccttgcacggaacaacaccattgtgaacgaattggtgcgagtgaccagcgaaggagctggacttcaactgcagaaggtcactgtgctcggagtggctaccgctcctcagcaagtgctgtcgaatggagtccccgtgtcaaactttacctactcccctgacactaaggtgctcgacatttgcgtgtccctcctgatgggagagcagttccttgtgtcctggtgttga

SEQ ID NO: 48 - DNA, 2652 bp, artificial
  hGAAwt-delta-42
gcacaccccgggcggccgcgagcagtgcccacacagtgcgacgtcccccccaacagccgcttcgattgcgcccctgacaaggccatcacccaggaacagtgcgaggcccgcggctgttgctacatccctgcaaagcaggggctgcagggagcccagatggggcagccctggtgcttcttcccacccagctaccccagctacaagctggagaacctgagctcctctgaaatgggctacacggccaccctgacccgtaccacccccaccttcttccccaaggacatcctgaccctgcggctggacgtgatgatggagactgagaaccgcctccacttcacgatcaaagatccagctaacaggcgctacgaggtgcccttggagaccccgcatgtccacagccgggcaccgtccccactctacagcgtggagttctccgaggagcccttcggggtgatcgtgcgccggcagctggacggccgcgtgctgctgaacacgacggtggcgcccctgttctttgcggaccagttccttcagctgtccacctcgctgccctcgcagtatatcacaggcctcgccgagcacctcagtcccctgatgctcagcaccagctggaccaggatcaccctgtggaaccgggaccttgcgcccacgcccggtgcgaacctctacgggtctcaccctttctacctggcgctggaggacggcgggtcggcacacggggtgttcctgctaaacagcaatgccatggatgtggtcctgcagccgagccctgcccttagctggaggtcgacaggtgggatcctggatgtctacatcttcctgggcccagagcccaagagcgtggtgcagcagtacctggacgttgtgggatacccgttcatgccgccatactggggcctgggcttccacctgtgccgctggggctactcctccaccgctatcacccgccaggtggtggagaacatgaccagggcccacttccccctggacgtccagtggaacgacctggactacatggactcccggagggacttcacgttcaacaaggatggcttccgggacttcccggccatggtgcaggagctgcaccagggcggccggcgctacatgatgatcgtggatcctgccatcagcagctcgggccctgccgggagctacaggccctacgacgagggtctgcggaggggggttttcatcaccaacgagaccggccagccgctgattgggaaggtatggcccgggtccactgccttccccgacttcaccaaccccacagccctggcctggtgggaggacatggtggctgagttccatgaccaggtgcccttcgacggcatgtggattgacatgaacgagccttccaacttcatcaggggctctgaggacggctgccccaacaatgagctggagaacccaccctacgtgcctggggtggttggggggaccctccaggcggccaccatctgtgcctccagccaccagtttctctccacacactacaacctgcacaacctctacggcctgaccgaagccatcgcctcccacagggcgctggtgaaggctcgggggacacgcccatttgtgatctcccgctcgacctttgctggccacggccgatacgccggccactggacgggggacgtgtggagctcctgggagcagctcgcctcctccgtgccagaaatcctgcagtttaacctgctgggggtgcctctggtcggggccgacgtctgcggcttcctgggcaacacctcagaggagctgtgtgtgcgctggacccagctgggggccttctaccccttcatgcggaaccacaacagcctgctcagtctgccccaggagccgtacagcttcagcgagccggcccagcaggccatgaggaaggccctcaccctgcgctacgcactcctcccccacctctacacactgttccaccaggcccacgtcgcgggggagaccgtggcccggcccctcttcctggagttccccaaggactctagcacctggactgtggaccaccagctcctgtggggggaggccctgctcatcaccccagtgctccaggccgggaaggccgaagtgactggctacttccccttgggcacatggtacgacctgcagacggtgccagtagaggcccttggcagcctcccacccccacctgcagctccccgtgagccagccatccacagcgaggggcagtgggtgacgctgccggcccccctggacaccatcaacgtccacctccgggctgggtacatcatccccctgcagggccctggcctcacaaccacagagtcccgccagcagcccatggccctggctgtggccctgaccaagggtggggaggcccgaggggagctgttctgggacgatggagagagcctggaagtgctggagcgaggggcctacacacaggtcatcttcctggccaggaataacacgatcgtgaatgagctggtacgtgtgaccagtgagggagctggcctgcagctgcagaaggtgactgtcctgggcgtggccacggcgccccagcaggtcctctccaacggtgtccctgtctccaacttcacctacagccccgacaccaaggtcctggacatctgtgtctcgctgttgatgggagagcagtttctcgtcagctggtgttag

SEQ ID NO: 49 - DNA, 2649 bp, artificial
  hGAAwt-delta-43
caccccgggcggccgcgagcagtgcccacacagtgcgacgtcccccccaacagccgcttcgattgcgcccctgacaaggccatcacccaggaacagtgcgaggcccgcggctgttgctacatccctgcaaagcaggggctgcagggagcccagatggggcagccctggtgcttcttcccacccagctaccccagctacaagctggagaacctgagctcctctgaaatgggctacacggccaccctgacccgtaccacccccaccttcttccccaaggacatcctgaccctgcggctggacgtgatgatggagactgagaaccgcctccacttcacgatcaaagatccagctaacaggcgctacgaggtgcccttggagaccccgcatgtccacagccgggcaccgtccccactctacagcgtggagttctccgaggagcccttcggggtgatcgtgcgccggcagctggacggccgcgtgctgctgaacacgacggtggcgcccctgttctttgcggaccagttccttcagctgtccacctcgctgccctcgcagtatatcacaggcctcgccgagcacctcagtcccctgatgctcagcaccagctggaccaggatcaccctgtggaaccgggaccttgcgcccacgcccggtgcgaacctctacgggtctcaccctttctacctggcgctggaggacggcgggtcggcacacggggtgttcctgctaaacagcaatgccatggatgtggtcctgcagccgagccctgcccttagctggaggtcgacaggtgggatcctggatgtctacatcttcctgggcccagagcccaagagcgtggtgcagcagtacctggacgttgtgggatacccgttcatgccgccatactggggcctgggcttccacctgtgccgctggggctactcctccaccgctatcacccgccaggtggtggagaacatgaccagggcccacttccccctggacgtccagtggaacgacctggactacatggactcccggagggacttcacgttcaacaaggatggcttccgggacttcccggccatggtgcaggagctgcaccagggcggccggcgctacatgatgatcgtggatcctgccatcagcagctcgggccctgccgggagctacaggccctacgacgagggtctgcggaggggggttttcatcaccaacgagaccggccagccgctgattgggaaggtatggcccgggtccactgccttccccgacttcaccaaccccacagccctggcctggtgggaggacatggtggctgagttccatgaccaggtgcccttcgacggcatgtggattgacatgaacgagccttccaacttcatcaggggctctgaggacggctgccccaacaatgagctggagaacccaccctacgtgcctggggtggttggggggaccctccaggcggccaccatctgtgcctccagccaccagtttctctccacacactacaacctgcacaacctctacggcctgaccgaagccatcgcctcccacagggcgctggtgaaggctcgggggacacgcccatttgtgatctcccgctcgacctttgctggccacggccgatacgccggccactggacgggggacgtgtggagctcctgggagcagctcgcctcctccgtgccagaaatcctgcagtttaacctgctgggggtgcctctggtcggggccgacgtctgcggcttcctgggcaacacctcagaggagctgtgtgtgcgctggacccagctgggggccttctaccccttcatgcggaaccacaacagcctgctcagtctgccccaggagccgtacagcttcagcgagccggcccagcaggccatgaggaaggccctcaccctgcgctacgcactcctcccccacctctacacactgttccaccaggcccacgtcgcgggggagaccgtggcccggcccctcttcctggagttccccaaggactctagcacctggactgtggaccaccagctcctgtggggggaggccctgctcatcaccccagtgctccaggccgggaaggccgaagtgactggctacttccccttgggcacatggtacgacctgcagacggtgccagtagaggcccttggcagcctcccacccccacctgcagctccccgtgagccagccatccacagcgaggggcagtgggtgacgctgccggcccccctggacaccatcaacgtccacctccgggctgggtacatcatccccctgcagggccctggcctcacaaccacagagtcccgccagcagcccatggccctggctgtggccctgaccaagggtggggaggcccgaggggagctgttctgggacgatggagagagcctggaagtgctggagcgaggggcctacacacaggtcatcttcctggccaggaataacacgatcgtgaatgagctggtacgtgtgaccagtgagggagctggcctgcagctgcagaaggtgactgtcctgggcgtggccacggcgccccagcaggtcctctccaacggtgtccctgtctccaacttcacctacagccccgacaccaaggtcctggacatctgtgtctcgctgttgatgggagagcagtttctcgtcagctggtgttag

SEQ ID NO: 50 - DNA, 2649 bp, artificial
  hGAAco1-delta-43
caccccggcagacctagagctgtgcctacccagtgtgacgtgccccccaacagcagattcgactgcgcccctgacaaggccatcacccaggaacagtgcgaggccagaggctgctgctacatccctgccaagcagggactgcagggcgctcagatgggacagccctggtgcttcttcccaccctcctaccccagctacaagctggaaaacctgagcagcagcgagatgggctacaccgccaccctgaccagaaccacccccacattcttcccaaaggacatcctgaccctgcggctggacgtgatgatggaaaccgagaaccggctgcacttcaccatcaaggaccccgccaatcggagatacgaggtgcccctggaaaccccccacgtgcactctagagcccccagccctctgtacagcgtggaattcagcgaggaacccttcggcgtgatcgtgcggagacagctggatggcagagtgctgctgaacaccaccgtggcccctctgttcttcgccgaccagttcctgcagctgagcaccagcctgcccagccagtacatcacaggactggccgagcacctgagccccctgatgctgagcacatcctggacccggatcaccctgtggaacagggatctggcccctacccctggcgccaatctgtacggcagccaccctttctacctggccctggaagatggcggatctgcccacggagtgtttctgctgaactccaacgccatggacgtggtgctgcagcctagccctgccctgtcttggagaagcacaggcggcatcctggatgtgtacatctttctgggccccgagcccaagagcgtggtgcagcagtatctggatgtcgtgggctaccccttcatgcccccttactggggcctgggattccacctgtgcagatggggctactccagcaccgccatcaccagacaggtggtggaaaacatgaccagagcccacttcccactggatgtgcagtggaacgacctggactacatggacagcagacgggacttcaccttcaacaaggacggcttccgggacttccccgccatggtgcaggaactgcatcagggcggcagacggtacatgatgatcgtggatcccgccatcagctcctctggccctgccggctcttacagaccctacgacgagggcctgcggagaggcgtgttcatcaccaacgagacaggccagcccctgatcggcaaagtgtggcctggcagcacagccttccccgacttcaccaatcctaccgccctggcttggtgggaggacatggtggccgagttccacgaccaggtgcccttcgacggcatgtggatcgacatgaacgagcccagcaacttcatccggggcagcgaggatggctgccccaacaacgaactggaaaatcccccttacgtgcccggcgtcgtgggcggaacactgcaggccgctacaatctgtgccagcagccaccagtttctgagcacccactacaacctgcacaacctgtacggcctgaccgaggccattgccagccaccgcgctctcgtgaaagccagaggcacacggcccttcgtgatcagcagaagcacctttgccggccacggcagatacgccggacattggactggcgacgtgtggtcctcttgggagcagctggcctctagcgtgcccgagatcctgcagttcaatctgctgggcgtgccactcgtgggcgccgatgtgtgtggcttcctgggcaacacctccgaggaactgtgtgtgcggtggacacagctgggcgccttctaccctttcatgagaaaccacaacagcctgctgagcctgccccaggaaccctacagctttagcgagcctgcacagcaggccatgcggaaggccctgacactgagatacgctctgctgccccacctgtacaccctgtttcaccaggcccatgtggccggcgagacagtggccagacctctgtttctggaattccccaaggacagcagcacctggaccgtggaccatcagctgctgtggggagaggctctgctgattaccccagtgctgcaggcaggcaaggccgaagtgaccggctactttcccctgggcacttggtacgacctgcagaccgtgcctgtggaagccctgggatctctgcctccacctcctgccgctcctagagagcctgccattcactctgagggccagtgggtcacactgcctgcccccctggataccatcaacgtgcacctgagggccggctacatcataccactgcagggacctggcctgaccaccaccgagtctagacagcagccaatggccctggccgtggccctgaccaaaggcggagaagctaggggcgagctgttctgggacgatggcgagagcctggaagtgctggaaagaggcgcctatacccaagtgatcttcctggcccggaacaacaccatcgtgaacgagctggtgcgcgtgacctctgaaggcgctggactgcagctgcagaaagtgaccgtgctgggagtggccacagcccctcagcaggtgctgtctaatggcgtgcccgtgtccaacttcacctacagccccgacaccaaggtgctggacatctgcgtgtcactgctgatgggagagcagtttctggtgtcctggtgctga

SEQ ID NO: 51 - DNA, 2649 bp, artificial
  hGAAco2-delta-43
catcctggtagaccaagagctgtgcctacccaatgcgacgtgccacccaactcccgattcgactgcgcgccagataaggctattacccaagagcagtgtgaagccagaggttgctgctacatcccagcgaagcaaggattgcaaggcgcccaaatgggacaaccttggtgtttcttccccccttcgtacccatcatataaactcgaaaacctgtcctcttcggaaatgggttatactgccaccctcaccagaactactcctactttcttcccgaaagacatcttgaccttgaggctggacgtgatgatggagactgaaaaccggctgcatttcactatcaaagatcctgccaatcggcgatacgaggtccctctggaaacccctcacgtgcactcacgggctccttctccgctttactccgtcgaattctctgaggaacccttcggagtgatcgttagacgccagctggatggtagagtgctgttgaacactactgtggccccacttttcttcgctgaccagtttctgcaactgtccacttccctgccatcccagtacattactggactcgccgaacacctgtcgccactgatgctctcgacctcttggactagaatcactttgtggaacagagacttggcccctactccgggagcaaatctgtacggaagccaccctttttacctggcgctcgaagatggcggatccgctcacggagtgttcctgctgaatagcaacgcaatggacgtggtgctgcaaccttcccctgcactcagttggagaagtaccgggggtattctggacgtgtacatcttcctcggaccagaacccaagagcgtggtgcagcaatatctggacgtggtcggatacccttttatgcctccttactggggactgggattccacctttgccgttggggctactcatccaccgccattaccagacaggtggtggagaatatgaccagagcccacttccctctcgacgtgcagtggaacgatctggactatatggactcccggagagatttcaccttcaacaaggacgggttccgcgattttcccgcgatggttcaagagctccaccagggtggtcgaagatatatgatgatcgtcgacccagccatttcgagcagcggacccgctggatcttatagaccttacgacgaaggccttaggagaggagtgttcatcacaaacgagactggacagcctttgatcggtaaagtgtggcctggatcaaccgcctttcctgactttaccaatcccactgccttggcttggtgggaggacatggtggccgaattccacgaccaagtcccctttgatggaatgtggatcgatatgaacgaaccaagcaattttatcagaggttccgaagacggttgccccaacaacgaactggaaaaccctccttatgtgcccggagtcgtgggcggaacattacaggccgcgactatttgcgccagcagccaccaattcctgtccactcactacaacctccacaacctttatggattaaccgaagctattgcaagtcacagggctctggtgaaggctagagggactaggccctttgtgatctcccgatccacctttgccggacacgggagatacgccggtcactggactggtgacgtgtggagctcatgggaacaactggcctcctccgtgccggaaatcttacagttcaaccttctgggtgtccctcttgtcggagcagacgtgtgtgggtttcttggtaacacctccgaggaactgtgtgtgcgctggactcaactgggtgcattctacccattcatgagaaaccacaactccttgctgtccctgccacaagagccctactcgttcagcgagcctgcacaacaggctatgcggaaggcactgaccctgagatacgccctgcttccacacttatacactctcttccatcaagcgcatgtggcaggagaaaccgttgcaaggcctcttttccttgaattccccaaggattcctcgacttggacggtggatcatcagctgctgtggggagaagctctgctgattactccagtgttgcaagccggaaaagctgaggtgaccggatactttccgctgggaacctggtacgacctccagactgtccctgttgaagcccttggatcactgcctccgcctccggcagctccacgcgaaccagctatacattccgagggacagtgggttacattaccagctcctctggacacaatcaacgtccacttaagagctggctacattatccctctgcaaggaccaggactgactacgaccgagagcagacagcagccaatggcactggctgtggctctgaccaagggaggggaagctagaggagaactcttctgggatgatggggagtcccttgaagtgctggaaagaggcgcttacactcaagtcattttccttgcacggaacaacaccattgtgaacgaattggtgcgagtgaccagcgaaggagctggacttcaactgcagaaggtcactgtgctcggagtggctaccgctcctcagcaagtgctgtcgaatggagtccccgtgtcaaactttacctactcccctgacactaaggtgctcgacatttgcgtgtccctcctgatgggagagcagttccttgtgtcctggtgttga

SEQ ID NO: 52 - DNA, 2637 bp, artificial
  hGAAwt-delta-47
ccgcgagcagtgcccacacagtgcgacgtcccccccaacagccgcttcgattgcgcccctgacaaggccatcacccaggaacagtgcgaggcccgcggctgttgctacatccctgcaaagcaggggctgcagggagcccagatggggcagccctggtgcttcttcccacccagctaccccagctacaagctggagaacctgagctcctctgaaatgggctacacggccaccctgacccgtaccacccccaccttcttccccaaggacatcctgaccctgcggctggacgtgatgatggagactgagaaccgcctccacttcacgatcaaagatccagctaacaggcgctacgaggtgcccttggagaccccgcatgtccacagccgggcaccgtccccactctacagcgtggagttctccgaggagcccttcggggtgatcgtgcgccggcagctggacggccgcgtgctgctgaacacgacggtggcgcccctgttctttgcggaccagttccttcagctgtccacctcgctgccctcgcagtatatcacaggcctcgccgagcacctcagtcccctgatgctcagcaccagctggaccaggatcaccctgtggaaccgggaccttgcgcccacgcccggtgcgaacctctacgggtctcaccctttctacctggcgctggaggacggcgggtcggcacacggggtgttcctgctaaacagcaatgccatggatgtggtcctgcagccgagccctgcccttagctggaggtcgacaggtgggatcctggatgtctacatcttcctgggcccagagcccaagagcgtggtgcagcagtacctggacgttgtgggatacccgttcatgccgccatactggggcctgggcttccacctgtgccgctggggctactcctccaccgctatcacccgccaggtggtggagaacatgaccagggcccacttccccctggacgtccagtggaacgacctggactacatggactcccggagggacttcacgttcaacaaggatggcttccgggacttcccggccatggtgcaggagctgcaccagggcggccggcgctacatgatgatcgtggatcctgccatcagcagctcgggccctgccgggagctacaggccctacgacgagggtctgcggaggggggttttcatcaccaacgagaccggccagccgctgattgggaaggtatggcccgggtccactgccttccccgacttcaccaaccccacagccctggcctggtgggaggacatggtggctgagttccatgaccaggtgcccttcgacggcatgtggattgacatgaacgagccttccaacttcatcaggggctctgaggacggctgccccaacaatgagctggagaacccaccctacgtgcctggggtggttggggggaccctccaggcggccaccatctgtgcctccagccaccagtttctctccacacactacaacctgcacaacctctacggcctgaccgaagccatcgcctcccacagggcgctggtgaaggctcgggggacacgcccatttgtgatctcccgctcgacctttgctggccacggccgatacgccggccactggacgggggacgtgtggagctcctgggagcagctcgcctcctccgtgccagaaatcctgcagtttaacctgctgggggtgcctctggtcggggccgacgtctgcggcttcctgggcaacacctcagaggagctgtgtgtgcgctggacccagctgggggccttctaccccttcatgcggaaccacaacagcctgctcagtctgccccaggagccgtacagcttcagcgagccggcccagcaggccatgaggaaggccctcaccctgcgctacgcactcctcccccacctctacacactgttccaccaggcccacgtcgcgggggagaccgtggcccggcccctcttcctggagttccccaaggactctagcacctggactgtggaccaccagctcctgtggggggaggccctgctcatcaccccagtgctccaggccgggaaggccgaagtgactggctacttccccttgggcacatggtacgacctgcagacggtgccagtagaggcccttggcagcctcccacccccacctgcagctccccgtgagccagccatccacagcgaggggcagtgggtgacgctgccggcccccctggacaccatcaacgtccacctccgggctgggtacatcatccccctgcagggccctggcctcacaaccacagagtcccgccagcagcccatggccctggctgtggccctgaccaagggtggggaggcccgaggggagctgttctgggacgatggagagagcctggaagtgctggagcgaggggcctacacacaggtcatcttcctggccaggaataacacgatcgtgaatgagctggtacgtgtgaccagtgagggagctggcctgcagctgcagaaggtgactgtcctgggcgtggccacggcgccccagcaggtcctctccaacggtgtccctgtctccaacttcacctacagccccgacaccaaggtcctggacatctgtgtctcgctgttgatgggagagcagtttctcgtcagctggtgttag

SEQ ID NO: 53 - DNA, 2637 bp, artificial
  hGAAco1-delta-47
cctagagctgtgcctacccagtgtgacgtgccccccaacagcagattcgactgcgcccctgacaaggccatcacccaggaacagtgcgaggccagaggctgctgctacatccctgccaagcagggactgcagggcgctcagatgggacagccctggtgcttcttcccaccctcctaccccagctacaagctggaaaacctgagcagcagcgagatgggctacaccgccaccctgaccagaaccacccccacattcttcccaaaggacatcctgaccctgcggctggacgtgatgatggaaaccgagaaccggctgcacttcaccatcaaggaccccgccaatcggagatacgaggtgcccctggaaaccccccacgtgcactctagagcccccagccctctgtacagcgtggaattcagcgaggaacccttcggcgtgatcgtgcggagacagctggatggcagagtgctgctgaacaccaccgtggcccctctgttcttcgccgaccagttcctgcagctgagcaccagcctgcccagccagtacatcacaggactggccgagcacctgagccccctgatgctgagcacatcctggacccggatcaccctgtggaacagggatctggcccctacccctggcgccaatctgtacggcagccaccctttctacctggccctggaagatggcggatctgcccacggagtgtttctgctgaactccaacgccatggacgtggtgctgcagcctagccctgccctgtcttggagaagcacaggcggcatcctggatgtgtacatctttctgggccccgagcccaagagcgtggtgcagcagtatctggatgtcgtgggctaccccttcatgcccccttactggggcctgggattccacctgtgcagatggggctactccagcaccgccatcaccagacaggtggtggaaaacatgaccagagcccacttcccactggatgtgcagtggaacgacctggactacatggacagcagacgggacttcaccttcaacaaggacggcttccgggacttccccgccatggtgcaggaactgcatcagggcggcagacggtacatgatgatcgtggatcccgccatcagctcctctggccctgccggctcttacagaccctacgacgagggcctgcggagaggcgtgttcatcaccaacgagacaggccagcccctgatcggcaaagtgtggcctggcagcacagccttccccgacttcaccaatcctaccgccctggcttggtgggaggacatggtggccgagttccacgaccaggtgcccttcgacggcatgtggatcgacatgaacgagcccagcaacttcatccggggcagcgaggatggctgccccaacaacgaactggaaaatcccccttacgtgcccggcgtcgtgggcggaacactgcaggccgctacaatctgtgccagcagccaccagtttctgagcacccactacaacctgcacaacctgtacggcctgaccgaggccattgccagccaccgcgctctcgtgaaagccagaggcacacggcccttcgtgatcagcagaagcacctttgccggccacggcagatacgccggacattggactggcgacgtgtggtcctcttgggagcagctggcctctagcgtgcccgagatcctgcagttcaatctgctgggcgtgccactcgtgggcgccgatgtgtgtggcttcctgggcaacacctccgaggaactgtgtgtgcggtggacacagctgggcgccttctaccctttcatgagaaaccacaacagcctgctgagcctgccccaggaaccctacagctttagcgagcctgcacagcaggccatgcggaaggccctgacactgagatacgctctgctgccccacctgtacaccctgtttcaccaggcccatgtggccggcgagacagtggccagacctctgtttctggaattccccaaggacagcagcacctggaccgtggaccatcagctgctgtggggagaggctctgctgattaccccagtgctgcaggcaggcaaggccgaagtgaccggctactttcccctgggcacttggtacgacctgcagaccgtgcctgtggaagccctgggatctctgcctccacctcctgccgctcctagagagcctgccattcactctgagggccagtgggtcacactgcctgcccccctggataccatcaacgtgcacctgagggccggctacatcataccactgcagggacctggcctgaccaccaccgagtctagacagcagccaatggccctggccgtggccctgaccaaaggcggagaagctaggggcgagctgttctgggacgatggcgagagcctggaagtgctggaaagaggcgcctatacccaagtgatcttcctggcccggaacaacaccatcgtgaacgagctggtgcgcgtgacctctgaaggcgctggactgcagctgcagaaagtgaccgtgctgggagtggccacagcccctcagcaggtgctgtctaatggcgtgcccgtgtccaacttcacctacagccccgacaccaaggtgctggacatctgcgtgtcactgctgatgggagagcagtttctggtgtcctggtgctga

SEQ ID NO: 54 - DNA, 2637 bp, artificial
  hGAAco2-delta-47
ccaagagctgtgcctacccaatgcgacgtgccacccaactcccgattcgactgcgcgccagataaggctattacccaagagcagtgtgaagccagaggttgctgctacatcccagcgaagcaaggattgcaaggcgcccaaatgggacaaccttggtgtttcttccccccttcgtacccatcatataaactcgaaaacctgtcctcttcggaaatgggttatactgccaccctcaccagaactactcctactttcttcccgaaagacatcttgaccttgaggctggacgtgatgatggagactgaaaaccggctgcatttcactatcaaagatcctgccaatcggcgatacgaggtccctctggaaacccctcacgtgcactcacgggctccttctccgctttactccgtcgaattctctgaggaacccttcggagtgatcgttagacgccagctggatggtagagtgctgttgaacactactgtggccccacttttcttcgctgaccagtttctgcaactgtccacttccctgccatcccagtacattactggactcgccgaacacctgtcgccactgatgctctcgacctcttggactagaatcactttgtggaacagagacttggcccctactccgggagcaaatctgtacggaagccaccctttttacctggcgctcgaagatggcggatccgctcacggagtgttcctgctgaatagcaacgcaatggacgtggtgctgcaaccttcccctgcactcagttggagaagtaccgggggtattctggacgtgtacatcttcctcggaccagaacccaagagcgtggtgcagcaatatctggacgtggtcggatacccttttatgcctccttactggggactgggattccacctttgccgttggggctactcatccaccgccattaccagacaggtggtggagaatatgaccagagcccacttccctctcgacgtgcagtggaacgatctggactatatggactcccggagagatttcaccttcaacaaggacgggttccgcgattttcccgcgatggttcaagagctccaccagggtggtcgaagatatatgatgatcgtcgacccagccatttcgagcagcggacccgctggatcttatagaccttacgacgaaggccttaggagaggagtgttcatcacaaacgagactggacagcctttgatcggtaaagtgtggcctggatcaaccgcctttcctgactttaccaatcccactgccttggcttggtgggaggacatggtggccgaattccacgaccaagtcccctttgatggaatgtggatcgatatgaacgaaccaagcaattttatcagaggttccgaagacggttgccccaacaacgaactggaaaaccctccttatgtgcccggagtcgtgggcggaacattacaggccgcgactatttgcgccagcagccaccaattcctgtccactcactacaacctccacaacctttatggattaaccgaagctattgcaagtcacagggctctggtgaaggctagagggactaggccctttgtgatctcccgatccacctttgccggacacgggagatacgccggtcactggactggtgacgtgtggagctcatgggaacaactggcctcctccgtgccggaaatcttacagttcaaccttctgggtgtccctcttgtcggagcagacgtgtgtgggtttcttggtaacacctccgaggaactgtgtgtgcgctggactcaactgggtgcattctacccattcatgagaaaccacaactccttgctgtccctgccacaagagccctactcgttcagcgagcctgcacaacaggctatgcggaaggcactgaccctgagatacgccctgcttccacacttatacactctcttccatcaagcgcatgtggcaggagaaaccgttgcaaggcctcttttccttgaattccccaaggattcctcgacttggacggtggatcatcagctgctgtggggagaagctctgctgattactccagtgttgcaagccggaaaagctgaggtgaccggatactttccgctgggaacctggtacgacctccagactgtccctgttgaagcccttggatcactgcctccgcctccggcagctccacgcgaaccagctatacattccgagggacagtgggttacattaccagctcctctggacacaatcaacgtccacttaagagctggctacattatccctctgcaaggaccaggactgactacgaccgagagcagacagcagccaatggcactggctgtggctctgaccaagggaggggaagctagaggagaactcttctgggatgatggggagtcccttgaagtgctggaaagaggcgcttacactcaagtcattttccttgcacggaacaacaccattgtgaacgaattggtgcgagtgaccagcgaaggagctggacttcaactgcagaaggtcactgtgctcggagtggctaccgctcctcagcaagtgctgtcgaatggagtccccgtgtcaaactttacctactcccctgacactaaggtgctcgacatttgcgtgtccctcctgatgggagagcagttccttgtgtcctggtgttga